European Patent Application EP 4 588 519 A2, published July 23, 2025. Title: Immuno-Based Botulinum Toxin Serotype A Activity Assays. Applicant: ALLERGAN, INC. Application EP. The sequence listing filed with the application follows.

SEQUENCE LISTING (148 sequences)

SEQ ID NO: 1 - protein, 1296 aa, Clostridium botulinum
MPFVNKQFNYKDPVNGVDIAYIKIPNAGQMQPVKAFKIHNKIWVIPERDTFTNPEEGDLNPPPEAKQVPVSYYDSTYLSTDNEKDNYLKGVTKLFERIYSTDLGRMLLTSIVRGIPFWGGSTIDTELKVIDTNCINVIQPDGSYRSEELNLVIIGPSADIIQFECKSFGHEVLNLTRNGYGSTQYIRFSPDFTFGFEESLEVDTNPLLGAGKFATDPAVTLAHELIHAGHRLYGIAINPNRVFKVNTNAYYEMSGLEVSFEELRTFGGHDAKFIDSLQENEFRLYYYNKFKDIASTLNKAKSIVGTTASLQYMKNVFKEKYLLSEDTSGKFSVDKLKFDKLYKMLTEIYTEDNFVKFFKVLNRKTYLNFDKAVFKINIVPKVNYTIYDGFNLRNTNLAANFNGQNTEINNMNFTKLKNFTGLFEFYKLLCVRGIITSKTKSLDKGYNKALNDLCIKVNNWDLFFSPSEDNFTNDLNKGEEITSDTNIEAAEENISLDLIQQYYLTFNFDNEPENISIENLSSDIIGQLELMPNIERFPNGKKYELDKYTMFHYLRAQEFEHGKSRIALTNSVNEALLNPSRVYTFFSSDYVKKVNKATEAAMFLGWVEQLVYDFTDETSEVSTTDKIADITIIIPYIGPALNIGNMLYKDDFVGALIFSGAVILLEFIPEIAIPVLGTFALVSYIANKVLTVQTIDNALSKRNEKWDEVYKYIVTNWLAKVNTQIDLIRKKMKEALENQAEATKAIINYQYNQYTEEEKNNINFNIDDLSSKLNESINKAMININKFLNQCSVSYLMNSMIPYGVKRLEDFDASLKDALLKYIYDNRGTLIGQVDRLKDKVNNTLSTDIPFQLSKYVDNQRLLSTFTEYIKNIINTSILNLRYESNHLIDLSRYASKINIGSKVNFDPIDKNQIQLFNLESSKIEVILKNAIVYNSMYENFSTSFWIRIPKYFNSISLNNEYTIINCMENNSGWKVSLNYGEIIWTLQDTQEIKQRVVFKYSQMINISDYINRWIFVTITNNRLNNSKIYINGRLIDQKPISNLGNIHASNNIMFKLDGCRDTHRYIWIKYFNLFDKELNEKEIKDLYDNQSNSGILKDFWGDYLQYDKPYYMLNLYDPNKYVDVNNVGIRGYMYLKGPRGSVMTTNIYLNSSLYRGTKFIIKKYASGNKDNIVRNNDRVYINVVVKNKEYRLATNASQAGVEKILSALEIPDVGNLSQVVVMKSKNDQGITNKCKMNLQDNNGNDIGFIGFHQFNNIAKLVASNWYNRQIERSSRTLGCSWEFIPVDDGWGERPL

SEQ ID NO: 2 - protein, 1296 aa, Clostridium botulinum
MPFVNKQFNYKDPVNGVDIAYIKIPNAGQMQPVKAFKIHNKIWVIPERDTFTNPEEGDLNPPPEAKQVPVSYYDSTYLSTDNEKDNYLKGVTKLFERIYSTDLGRMLLTSIVRGIPFWGGSTIDTELKVIDTNCINVIQPDGSYRSEELNLVIIGPSADIIQFECKSFGHDVLNLTRNGYGSTQYIRFSPDFTFGFEESLEVDTNPLLGAGKFATDPAVTLAHELIHAEHRLYGIAINPNRVFKVNTNAYYEMSGLEVSFEELRTFGGHDAKFIDSLQENEFRLYYYNKFKDVASTLNKAKSIIGTTASLQYMKNVFKEKYLLSEDTSGKFSVDKLKFDKLYKMLTEIYTEDNFVNFFKVINRKTYLNFDKAVFRINIVPDENYTIKDGFNLKGANLSTNFNGQNTEINSRNFTRLKNFTGLFEFYKLLCVRGIIPFKTKSLDEGYNKALNDLCIKVNNWDLFFSPSEDNFTNDLDKVEEITADTNIEAAEENISLDLIQQYYLTFDFDNEPENISIENLSSDIIGQLEPMPNIERFPNGKKYELDKYTMFHYLRAQEFEHGDSRIILTNSAEEALLKPNVAYTFFSSKYVKKINKAVEAFMFLNWAEELVYDFTDETNEVTTMDKIADITIIVPYIGPALNIGNMLSKGEFVEAIIFTGVVAMLEFIPEYALPVFGTFAIVSYIANKVLTVQTINNALSKRNEKWDEVYKYTVTNWLAKVNTQIDLIREKMKKALENQAEATKAIINYQYNQYTEEEKNNINFNIDDLSSKLNESINSAMININKFLDQCSVSYLMNSMIPYAVKRLKDFDASVRDVLLKYIYDNRGTLVLQVDRLKDEVNNTLSADIPFQLSKYVDNKKLLSTFTEYIKNIVNTSILSIVYKKDDLIDLSRYGAKINIGDRVYYDSIDKNQIKLINLESSTIEVILKNAIVYNSMYENFSTSFWIKIPKYFSKINLNNEYTIINCIENNSGWKVSLNYGEIIWTLQDNKQNIQRVVFKYSQMVNISDYINRWIFVTITNNRLTKSKIYINGRLIDQKPISNLGNIHASNKIMFKLDGCRDPRRYIMIKYFNLFDKELNEKEIKDLYDSQSNSGILKDFWGNYLQYDKPYYMLNLFDPNKYVDVNNIGIRGYMYLKGPRGSVVTTNIYLNSTLYEGTKFIIKKYASGNEDNIVRNNDRVYINVVVKNKEYRLATNASQAGVEKILSALEIPDVGNLSQVVVMKSKDDQGIRNKCKMNLQDNNGNDIGFIGFHLYDNIAKLVASNWYNRQVGKASRTFGCSWEFIPVDDGWGESSL

SEQ ID NO: 3 - protein, 1292 aa, Clostridium botulinum
MPFVNKPFNYRDPGNGVDIAYIKIPNAGQMQPVKAFKIHEGVWVIPERDTFTNPEEGDLNPPPEAKQVPVSYYDSTYLSTDNEKDNYLKGVIKLFDRIYSTGLGRMLLSFIVKGIPFWGGSTIDTELKVIDTNCINVIEPGGSYRSEELNLVITGPSADIIQFECKSFGHDVFNLTRNGYGSTQYIRFSPDFTFGFEESLEVDTNPLLGAGTFATDPAVTLAHELIHAAHRLYGIAINPNRVLKVKTNAYYEMSGLEVSFEELRTFGGNDTNFIDSLWQKKFSRDAYDNLQNIARILNEAKTIVGTTTPLQYMKNIFIRKYFLSEDASGKISVNKAAFKEFYRVLTRGFTELEFVNPFKVINRKTYLNFDKAVFRINIVPDENYTINEGFNLEGANSNGQNTEINSRNFTRLKNFTGLFEFYKLLCVRGIIPFKTKSLDEGYNKALNYLCIKVNNWDLFFSPSEDNFTNDLDKVEEITADTNIEAAEENISSDLIQQYYLTFDFDNEPENISIENLSSDIIGQLEPMPNIERFPNGKKYELDKYTMFHYLRAQEFEHGDSRIILTNSAEEALLKPNVAYTFFSSKYVKKINKAVEAVIFLSWAEELVYDFTDETNEVTTMDKIADITIIVPYIGPALNIGNMVSKGEFVEAILFTGVVALLEFIPEYSLPVFGTFAIVSYIANKVLTVQTINNALSKRNEKWDEVYKYTVTNWLAKVNTQIDLIREKMKKALENQAEATRAIINYQYNQYTEEEKNNINFNIDDLSSKLNRSINRAMININKFLDQCSVSYLMNSMIPYAVKRLKDFDASVRDVLLKYIYDNRGTLILQVDRLKDEVNNTLSADIPFQLSKYVNDKKLLSTFTEYIKNIVNTSILSIVYKKDDLIDLSRYGAKINIGDRVYYDSIDKNQIKLINLESSTIEVILKNAIVYNSMYENFSTSFWIKIPKYFSKINLNNEYTIINCIENNSGWKVSLNYGEIIWTLQDNKQNIQRVVFKYSQMVNISDYINRWMFVTITNNRLTKSKIYINGRLIDQKPISNLGNIHASNKIMFKLDGCRDPRRYIMIKYFNLFDKELNEKEIKDLYDSQSNPGILKDFWGNYLQYDKPYYMLNLFDPNKYVDVNNIGIRGYMYLKGPRGSVMTTNIYLNSTLYMGTKFIIKKYASGNEDNIVRNNDRVYINVVVKNKEYRLATNASQAGVEKILSALEIPDVGNLSQVVVMKSKDDQGIRNKCKMNLQDNNGNDIGFVGFHLYDNIAKLVASNWYNRQVGKASRTFGCSWEFIPVDDGWGESSL

SEQ ID NO: 4 - protein, 1296 aa, Clostridium botulinum
MPLVNQQINYYDPVNGVDIAYIKIPNAGKMQPVKAFKIHNKVWVIPERDIFTNPEEVDLNPPPEAKQVPISYYDSAYLSTDNEKDNYLKGVIKLFERIYSTDLGRMLLISIVRGIPFWGGGKIDTELKVIDTNCINIIQLDDSYRSEELNLAIIGPSANIIESQCSSFRDDVLNLTRNGYGSTQYIRFSPDFTVGFEESLEVDTNPLLGAGKFAQDPAVALAHELIHAEHRLYGIAINTNRVFKVNTNAYYEMAGLEVSLEELITFGGNDAKFIDSLQKKEFSLYYYNKFKDIASTLNKAKSIVGTTASLQYMKNVFKEKYLLSEDATGKFLVDRLKFDELYKLLTEIYTEDNFVKFFKVLNRKTYLNFDKAVFKINIVPDVNYTIHDGFNLRNTNLAANFNGQNIEINNKNFDKLKNFTGLFEFYKLLCVRGIITSKTKSLDEGYNKALNELCIKVNNWDLFFSPSEDNFTNDLDKVEEITSDTNIEAAEENISLDLIQQYYLNFNFDNEPENTSIENLSSDIIGQLEPMPNIERFPNGKKYELNKYTMFHYLRAQEFKHSNSRIILTNSAKEALLKPNIVYTFFSSKYIKAINKAVEAVTFVNWIENLVYDFTDETNEVSTMDKIADITIVIPYIGPALNIGNMIYKGEFVEAIIFSGAVILLEIVPEIALPVLGTFALVSYVSNKVLTVQTIDNALSKRNEKWDEVYKYIVTNWLAIVNTQINLIREKMKKALENQAEATKAIINYQYNQYTEEEKNNINFNIDDLSSKLNESINSAMININKFLDQCSVSYLMNSMIPYAVKRLKDFDASVRDVLLKYIYDNRGTLIGQVNRLKDKVNNTLSADIPFQLSKYVDNKKLLSTFTEYIKNITNASILSIVYKDDDLIDLSRYGAEIYNGDKVYYNSIDKNQIRLINLESSTIEVILKKAIVYNSMYENFSTSFWIRIPKYFNSISLNNEYTIINCMENNSGWKVSLNYGEIIWTFQDTQEIKQRVVFKYSQMINISDYINRWIFVTITNNRITKSKIYINGRLIDQKPISNLGNIHASNKIMFKLDGCRDPHRYIVIKYFNLFDKELSEKEIKDLYDNQSNSGILKDFWGDYLQYDKSYYMLNLYDPNKYVDVNNVGIRGYMYLKGPRDNVMTTNIYLNSSLYMGTKFIIKKYASGNKDNIVRNNDRVYINVVVKNKEYRLATNASQAGVEKILSALEIPDVGNLSQVVVMKSKNDQGITNKCKMNLQDNNGNDIGFIGFHQFNNIAKLVASNWYNRQIERSSRTLGCSWEFIPVDDGWRERPL

SEQ ID NO: 5 - protein, 206 aa, Homo sapiens
MAEDADMRNELEEMQRRADQLADESLESTRRMLQLVEESKDAGIRTLVMLDEQGEQLDRVEEGMNHINQDMKEAEKNLKDLGKCCGLFICPCNKLKSSDAYKKAWGNNQDGVVASQPARVVDEREQMAISGGFIRRVTNDARENEMDENLEQVSGIIGNLRHMALDMGNEIDTQNRQIDRIMEKADSNKTRIDEANQRATKMLGSG

SEQ ID NO: 6 - protein, 206 aa, Homo sapiens
MAEDADMRNELEEMQRRADQLADESLESTRRMLQLVEESKDAGIRTLVMLDEQGEQLERIEEGMDQINKDMKEAEKNLTDLGKFCGLCVCPCNKLKSSDAYKKAWGNNQDGVVASQPARVVDEREQMAISGGFIRRVTNDARENEMDENLEQVSGIIGNLRHMALDMGNEIDTQNRQIDRIMEKADSNKTRIDEANQRATKMLGSG

SEQ ID NO: 7 - protein, 206 aa, Macaca mulatta; identical to SEQ ID NO: 6

SEQ ID NO: 8 - protein, 206 aa, Rattus norvegicus; identical to SEQ ID NO: 5

SEQ ID NO: 9 - protein, 206 aa, Rattus norvegicus; identical to SEQ ID NO: 6

SEQ ID NO: 10 - protein, 206 aa, Mus musculus; identical to SEQ ID NO: 6

SEQ ID NO: 11 - protein, 206 aa, Gallus gallus; identical to SEQ ID NO: 6

SEQ ID NO: 12 - protein, 204 aa, Carassius auratus
MAEDADMRNELSDMQQRADQLADESLESTRRMLQLVEESKDAGIRTLVMLDEQGEQLERIEEGMDQINKDMKDAEKNLNDLGKFCGLCSCPCNKMKSGGSKAWGNNQDGVVASQPARVVDEREQMAISGGFIRRVTDDARENEMDENLEQVGGIIGNLRHMALDMGNEIDTQNRQIDRIMEKADSNKTRIDEANQRATKMLGSG

SEQ ID NO: 13 - protein, 203 aa, Carassius auratus
MADEADMRNELTDMQARADQLGDESLESTRRMLQLVEESKDAGIRTLVMLDEQGEQLERIEEGMDQINKDMKEAEKNLTDLGNLCGLCPCPCNKLKGGGQSWGNNQDGVVSSQPARVVDEREQMAISGGFIRRVTNDARENEMDENLEQVGSIIGNLRHMALDMGNEIDTQNRQIDRIMDMADSNKTRIDEANQRATKMLGSG

SEQ ID NO: 14 - protein, 204 aa, Danio rerio
MAEDSDMRNELADMQQRADQLADESLESTRRMLQLVEESKDAGIRTLVMLDEQGEQLERIEEGMDQINKDMKDAEKNLNDLGKFCGLCSCPCNKMKSGASKAWGNNQDGVVASQPARVVDEREQMAISGGFIRRVTDDARENEMDENLEQVGGIIGNLRHMALDMGNEIDTQNRQIDRIMEKADSNKTRIDEANQRATKMLGSG

SEQ ID NO: 15 - protein, 203 aa, Danio rerio
MADESDMRNELNDMQARADQLGDESLESTRRMLQLVEESKDAGIRTLVMLDEQGEQLERIEEGMDQINKDMKEAEKNLTDLGNLCGLCPCPCNKLKGGGQSWGNNQDGVVSSQPARVVDEREQMAISGGFIRRVTNDARENEMDENLEQVGSIIGNLRHMALDMGNEIDTQNRQIDRIMDMADSNKTRIDEANQRATKMLGSG

SEQ ID NO: 16 - protein, 210 aa, Torpedo marmorata
MENSVENSMDPRSEQEEMQRCADQITDESLESTRRMLQLVEESKDAGIRTLVMLDEQGEQLERIEEGMDQINKDMKEAEKNLSDLGKCCGLCSCPCNKLKNFEAGGAYKKVWGNNQDGVVASQPARVMDDREQMAMSGGYIRRITDDARENEMEENLDQVGSIIGNLRHMALDMSNEIGSQNAQIDRIVVKGDMNKARIDEANKHATKML

SEQ ID NO: 17 - protein, 206 aa, Xenopus laevis
MADDADMRNELEEMQRRADQLADESLESTRRMLQYVEGSKDAGIRTLVMLDEQGEQLDRVEEGMNHINQDMKEAEKNLKDLGKCCGLFICPCNKLKSSGAYNKAWGNNQDGVVASQPARVVDEREQMAISGGFVRRVTNDARETEMDENLEQVGGIIGNLRHMALDMGNEIDTQNRQIDRIMEKADSNKARIDEANKHATKMLGSG

SEQ ID NO: 18 - protein, 206 aa, Xenopus laevis
MADDADMRNELEEMQRRADQLADESLESTRRMLQYVEGSKDAGIRTLVMLDEQGEQLERIEEGMEQINKDMKEAEKNLTDLGKFCGLCVCPCNKLKSSDAYKKAWGNNQDGVVASQPARVVDEREQMAISGGFVRRVTNDARETEMDENLEQVGGIIGNLRHMALDMGNEIDTQNRQIDRIMEKADSNKARIDEANKHATKMLGSG

SEQ ID NO: 19 - protein, 212 aa, Strongylocentrotus purpuratus
MEDQNDMNMRSELEEIQMQSNMQTDESLESTRRMLQMAEESQDMGIKTLVMLDEQGEQLDRIEEGMDQINTDMREAEKNLTGLEKCCGICVCPWKKLGNFEKGDDYKKTWKGNDDGKVNSHQPMRMEDDRDGCGGNASMITRITNDAREDEMDENLTQVSSIVGNLRHMAIDMQSEIGAQNSQVGRITSKAESNEGRINSADKRAKNILRNK

SEQ ID NO: 20 - protein, 212 aa, Drosophila melanogaster
MPADPSEEVAPQVPKTELEELQINAQGVADESLESTRRMLALCEESKEAGIRTLVALDDQGEQLDRIEEGMDQINADMREAEKNLSGMEKCCGICVLPCNKSQSFKEDDGTWKGNDDGKVVNNQPQRVMDDRNGMMAQAGYIGRITNDAREDEMEENMGQVNTMIGNLRNMALDMGSELENQNRQIDRINRKGESNEARIAVANQRAHQLLK

SEQ ID NO: 21 - protein, 212 aa, Hirudo medicinalis
MAKDIKPKPANGRDSPTDLQEIQLQMNAITDDSLESTRRMLAMCEESKDAGIRTLVMLDEQGEQLDRIEEGMDQINQDMRDAEKNLEGMEKCCGLCILPWKRTKNFDKGAEWNKGDEGKVNTDGPRLVVGDGNMGPSGGFITKITNDAREEEMEQNMGEVSNMISNLRNMAVDMGSEIDSQNRQVDRINNKMTSNQLRISDANKRASKLLKE

SEQ ID NO: 22 - protein, 212 aa, Loligo pealei
MSANGEVEVPKTELEEIQQQCNQVTDDSLESTRRMLNMCEESKEAGIRTLVMLDEQGEQLDRIEEGLDQINQDMKDAEKNLEGMEKCCGLCVLPWKRGKSFEKSGDYANTWKKDDDGPTNTNGPRVTVGDQNGMGPSSGYVTRITNDAREDDMENNMKEVSSMIGNLRNMAIDMGNEIGSQNRQVDRIQQKAESNESRIDEANKKATKLLKN

SEQ ID NO: 23 - protein, 220 aa, Lymnaea stagnalis
MTTNGEILPVGEEEEEELGEDALLRKQIDCNTNESLESTRRMLSLCEESKEAGIKTLVMLDEQGEQLDRIEEGMGQINQDMRDAEKNLEGLEKCCGLCVLPWKRSKNFEKGSDYNKTWKASEDGKINTNGPRLVVDQGNGSGPTGGYITRITNDAREDEMEQNIGEVAGMVSNLRNMAVDMGNEIESQNKQLDRINQKGGSLNVRVDEANKRANRILRKQ

SEQ ID NO: 24 - protein, 207 aa, Caenorhabditis elegans
MSGDDDIPEGLEAINLKMNATTDDSLESTRRMLALCEESKEAGIKTLVMLDDQGEQLERCEGALDTINQDMKEAEDHLKGMEKCCGLCVLPWNKTDDFEKTEFAKAWKKDDDGGVISDQPRITVGDSSMGPQGGYITKITNDAREDEMDENVQQVSTMVGNLRNMAIDMSTEVSNQNRQLDRIHDKAQSNEVRVESANKRAKNLITK

SEQ ID NO: 25 - protein, 808 aa, Homo sapiens
MGAPACALALCVAVAIVAGASSESLGTEQRVVGRAAEVPGPEPGQQEQLVFGSGDAVELSCPPPGGGPMGPTVWVKDGTGLVPSERVLVGPQRLQVLNASHEDSGAYSCRQRLTQRVLCHFSVRVTDAPSSGDDEDGEDEAEDTGVDTGAPYWTRPERMDKKLLAVPAANTVRFRCPAAGNPTPSISWLKNGREFRGEHRIGGIKLRHQQWSLVMESVVPSDRGNYTCVVENKFGSIRQTYTLDVLERSPHRPILQAGLPANQTAVLGSDVEFHCKVYSDAQPHIQWLKHVEVNGSKVGPDGTPYVTVLKSWISESVEADVRLRLANVSERDGGEYLCRATNFIGVAEKAFWLSVHGPRAAEEELVEADEAGSVYAGILSYGVGFFLFILVVAAVTLCRLRSPPKKGLGSPTVHKISRFPLKRQVSLESNASMSSNTPLVRIARLSSGEGPTLANVSELELPADPKWELSRARLTLGKPLGEGCFGQVVMAEAIGIDKDRAAKPVTVAVKMLKDDATDKDLSDLVSEMEMMKMIGKHKNIINLLGACTQGGPLYVLVEYAAKGNLREFLRARRPPGLDYSFDTCKPPEEQLTFKDLVSCAYQVARGMEYLASQKCIHRDLAARNVLVTEDNVMKIADFGLARDVHNLDYYKKTTNGRLPVKWMAPEALFDRVYTHQSDVWSFGVLLWEIFTLGGSPYPGIPVEELFKLLKEGHRMDKPANCTHDLYMIMRECWHAAPSQRPTFKQLVEDLDRVLTVTSTDEYLDLSAPFEQYSPGGQDTPSSSSSGDDSVFAHDLLPPAPPSSGGSRT

SEQ ID NO: 26 - protein, 806 aa, Homo sapiens
MGAPACALALCVAVAIVAGASSESLGTEQRVVGRAAEVPGPEPGQQEQLVFGSGDAVELSCPPPGGGPMGPTVWVKDGTGLVPSERVLVGPQRLQVLNASHEDSGAYSCRQRLTQRVLCHFSVRVTDAPSSGDDEDGEDEAEDTGVDTGAPYWTRPERMDKKLLAVPAANTVRFRCPAAGNPTPSISWLKNGREFRGEHRIGGIKLRHQQWSLVMESVVPSDRGNYTCVVENKFGSIRQTYTLDVLERSPHRPILQAGLPANQTAVLGSDVEFHCKVYSDAQPHIQWLKHVEVNGSKVGPDGTPYVTVLKTAGANTTDKELEVLSLHNVTFEDAGEYTCLAGNSIGFSHHSAWLVVLPAEEELVEADEAGSVYAGILSYGVGFFLFILVVAAVTLCRLRSPPKKGLGSPTVHKISRFPLKRQVSLESNASMSSNTPLVRIARLSSGEGPTLANVSELELPADPKWELSRARLTLGKPLGEGCFGQVVMAEAIGIDKDRAAKPVTVAVKMLKDDATDKDLSDLVSEMEMMKMIGKHKNIINLLGACTQGGPLYVLVEYAAKGNLREFLRARRPPGLDYSFDTCKPPEEQLTFKDLVSCAYQVARGMEYLASQKCIHRDLAARNVLVTEDNVMKIADFGLARDVHNLDYYKKTTNGRLPVKWMAPEALFDRVYTHQSDVWSFGVLLWEIFTLGGSPYPGIPVEELFKLLKEGHRMDKPANCTHDLYMIMRECWHAAPSQRPTFKQLVEDLDRVLTVTSTDEYLDLSAPFEQYSPGGQDTPSSSSSGDDSVFAHDLLPPAPPSSGGSRT

SEQ ID NO: 27 - protein, 694 aa, Homo sapiens
MGAPACALALCVAVAIVAGASSESLGTEQRVVGRAAEVPGPEPGQQEQLVFGSGDAVELSCPPPGGGPMGPTVWVKDGTGLVPSERVLVGPQRLQVLNASHEDSGAYSCRQRLTQRVLCHFSVRVTDAPSSGDDEDGEDEAEDTGVDTGAPYWTRPERMDKKLLAVPAANTVRFRCPAAGNPTPSISWLKNGREFRGEHRIGGIKLRHQQWSLVMESVVPSDRGNYTCVVENKFGSIRQTYTLDVLERSPHRPILQAGLPANQTAVLGSDVEFHCKVYSDAQPHIQWLKHVEVNGSKVGPDGTPYVTVLKVSLESNASMSSNTPLVRIARLSSGEGPTLANVSELELPADPKWELSRARLTLGKPLGEGCFGQVVMAEAIGIDKDRAAKPVTVAVKMLKDDATDKDLSDLVSEMEMMKMIGKHKNIINLLGACTQGGPLYVLVEYAAKGNLREFLRARRPPGLDYSFDTCKPPEEQLTFKDLVSCAYQVARGMEYLASQKCIHRDLAARNVLVTEDNVMKIADFGLARDVHNLDYYKKTTNGRLPVKWMAPEALFDRVYTHQSDVWSFGVLLWEIFTLGGSPYPGIPVEELFKLLKEGHRMDKPANCTHDLYMIMRECWHAAPSQRPTFKQLVEDLDRVLTVTSTDEYLDLSAPFEQYSPGGQDTPSSSSSGDDSVFAHDLLPPAPPSSGGSRT

SEQ ID NO: 28 - protein, 604 aa, Homo sapiens
AQRRKEREELAQQYEAILRECGHGRFQWTLYFVLGLALMADGVEVFVVGFVLPSAEKDMCLSDSNKGMLGLIVYLGMMVGAFLWGGLADRLGRRQCLLISLSVNSVFAFFSSFVQGYGTFLFCRLLSGVGIGGSIPIVFSYFSEFLAQEKRGEHLSWLCMFWMIGGVYAAAMAWAIIPHYGWSFQMGSAYQFHSWRVFVLVCAFPSVFAIGALTTQPESPRFFLENGKHDEAWMVLKQVHDTNMRAKGHPERVFSVTHIKTIHQEDELIEIQSDTGTWYQRWGVRALSLGGQVWGNFLSCFGPEYRRITLMMMGVWFTMSFSYYGLTVWFPDMIRHLQAVDYASRTKVFPGERVEHVTFNFTLENQIHRGGQYFNDKFIGLRLKSVSFEDSLFEECYFEDVTSSNTFFRNCTFINTVFYNTDLFEYKFVNSRLINSTFLHNKEGCPLDVTGTGEGAYMVYFVSFLGTLAVLPGNIVSALLMDKIGRLRMLAGSSVMSCVSCFFLSFGNSESAMIALLCLFGGVSIASWNALDVLTVELYPSDKRTTAFGFLNALCKLAAVLGISIFTSFVGITKAAPILFASAALALGSSLALKLPETRGQVLQ

SEQ ID NO: 29 - protein, 683 aa, Homo sapiens [sequence omitted]

SEQ ID NO: 30 - protein, 727 aa, Homo sapiens
MEDSYKDRTSLMKGAKDIAREVKKQTVKKVNQAVDRAQDEYTQRSYSRFQDEEDDDDYYPAGETYNGEANDDEGSSEATEGHDEDDEIYEGEYQGIPSMNQAKDSIVSVGQPKGDEYKDRRELESERRADEEELAQQYELIIQECGHGRFQWALFFVLGMALMADGVEVFVVGFVLPSAETDLCIPNSGSGWLGSIVYLGMMVGAFFWGGLADKVGRKQSLLICMSVNGFFAFLSSFVQGYGFFLFCRLLSGFGIGGAIPTVFSYFAEVLAREKRGEHLSWLCMFWMIGGIYASAMAWAIIPHYGWSFSMGSAYQFHSWRVFVIVCALPCVSSVVALTFMPESPRFLLEVGKHDEAWMILKLIHDTNMRARGQPEKVFTVNKIKTPKQIDELIEIESDTGTWYRRCFVRIRTELYGIWLTFMRCFNYPVRDNTIKLTIVWFTLSFGYYGLSVWFPDVIKPLQSDEYALLTRNVERDKYANFTINFTMENQIHTGMEYDNGRFIGVKFKSVTFKDSVFKSCTFEDVTSVNTYFKNCTFIDTVFDNTDFEPYKFIDSEFKNCSFFHNKTGCQITFDDDYSAYWIYFVNFLGTLAVLPGNIVSALLMDRIGRLTMLGGSMVLSGISCFFLWFGTSESMMIGMLCLYNGLTISAWNSLDVVTVELYPTDRRATGFGFLNALCKAAAVLGNLIFGSLVSITKSIPILLASTVLVCGGLVGLCLPDTRTQVLM

SEQ ID NO: 31 - protein, 742 aa, Homo sapiens
MEEGFRDRAAFIRGAKDIAKEVKKHAAKKVVKGLDRVQDEYSRRSYSRFEEEDDDDDFPAPSDGYYRGEGTQDEEEGGASSDATEGHDEDDEIYEGEYQDIPRAESGGKGERMADGAPLAGVRGGLSDGEGPPGGRGEAQRRKEREELAQQYEAILRECGHGRFQWTLYFVLGLALMADGVEVFVVGFVLPSAEKDMCLSDSNKGMLGLIVYLGMMVGAFLWGGLADRLGRRQCLLISLSVNSVFAFFSSFVQGYGTFLFCRLLSGVGIGGSIPIVFSYFSEFLAQEKRGEHLSWLCMFWMIGGVYAAAMAWAIIPHYGWSFQMGSAYQFHSWRVFVLVCAFPSVFAIGALTTQPESPRFFLENGKHDEAWMVLKQVHDTNMRAKGHPERVFSVTHIKTIHQEDELIEIQSDTGTWYQRWGVRALSLGGQVWGNFLSCFGPEYRRITLMMMGVWFTMSFSYYGLTVWFPDMIRHLQAVDYASRTKVFPGERVGHVTFNFTLENQIHRGGQYFNDKFIGLRLKSVSFEDSLFEECYFEDVTSSNTFFRNCTFINTVFYNTDLFEYKFVNSRLINSTFLHNKEGCPLDVTGTGEGAYMVYFVSFLGTLAVLPGNIVSALLMDKIGRLRMLAGSSVMSCVSCFFLSFGNSESAMIALLCLFGGVSIASWNALDVLTVELYPSDKRTTAFGFLNALCKLAAVLGISIFTSFVGITKAAPILFASAALALGSSLALKLPETRGQVLQ

SEQ ID NO: 32 - protein, 7 aa, synthetic construct
  REGION 1..7: note = SNAP-25 antigen having a free carboxyl-terminus atthe P1 residue of the scissile bond of the BoNT/Acleavage site
RIDEANQ

SEQ ID NO: 33 - protein, 8 aa, synthetic construct
  REGION 1..8: note = SNAP-25 antigen having a free carboxyl-terminus atthe P1 residue of the scissile bond of the BoNT/Acleavage site
TRIDEANQ

SEQ ID NO: 34 - protein, 9 aa, synthetic construct
  REGION 1..9: note = SNAP-25 antigen having a free carboxyl-terminus atthe P1 residue of the scissile bond of the BoNT/Acleavage site
KTRIDEANQ

SEQ ID NO: 35 - protein, 10 aa, synthetic construct
  REGION 1..10: note = SNAP-25 antigen having a free carboxyl-terminus atthe P1 residue of the scissile bond of the BoNT/Acleavage site
NKTRIDEANQ

SEQ ID NO: 36 - protein, 11 aa, synthetic construct
  REGION 1..11: note = SNAP-25 antigen having a free carboxyl-terminus atthe P1 residue of the scissile bond of the BoNT/Acleavage site
SNKTRIDEANQ

SEQ ID NO: 37 - protein, 12 aa, synthetic construct
  REGION 1..12: note = SNAP-25 antigen having a free carboxyl-terminus atthe P1 residue of the scissile bond of the BoNT/Acleavage site
DSNKTRIDEANQ

SEQ ID NO: 38 - protein, 13 aa, synthetic construct
  SITE 13: note = SNAP-25 antigen having a free carboxylatedcarboxyl-terminus at the P1 residue of thescissile bond of the BoNT/A cleavage site, carboxylated glutamine
CDSNKTRIDEANQ

SEQ ID NO: 39 - protein, 7 aa, synthetic construct
  REGION 1..7: note = SNAP-25 antigen having a free carboxyl-terminus atthe P1 residue of the scissile bond of the BoNT/Acleavage site
RIDEANK

SEQ ID NO: 40 - protein, 8 aa, synthetic construct
  REGION 1..8: note = SNAP-25 antigen having a free carboxyl-terminus atthe P1 residue of the scissile bond of the BoNT/Acleavage site
ARIDEANK

SEQ ID NO: 41 - protein, 9 aa, synthetic construct
  REGION 1..9: note = SNAP-25 antigen having a free carboxyl-terminus atthe P1 residue of the scissile bond of the BoNT/Acleavage site
KARIDEANK

SEQ ID NO: 42 - protein, 10 aa, synthetic construct
  REGION 1..10: note = SNAP-25 antigen having a free carboxyl-terminus atthe P1 residue of the scissile bond of the BoNT/Acleavage site
NKARIDEANK

SEQ ID NO: 43 - protein, 11 aa, synthetic construct
  REGION 1..11: note = SNAP-25 antigen having a free carboxyl-terminus atthe P1 residue of the scissile bond of the BoNT/Acleavage site
MNKARIDEANK

SEQ ID NO: 44 - protein, 12 aa, synthetic construct
  REGION 1..12: note = SNAP-25 antigen having a free carboxyl-terminus atthe P1 residue of the scissile bond of the BoNT/Acleavage site
DMNKARIDEANK

SEQ ID NO: 45 - protein, 13 aa, synthetic construct
  SITE 13: note = SNAP-25 antigen having a free carboxylatedcarboxyl-terminus at the P1 residue of thescissile bond of the BoNT/A cleavage site, Carboxylated lysine
CDMNKARIDEANK

SEQ ID NO: 46 - protein, 11 aa, synthetic construct
  REGION 1..11: note = SNAP-25 antigen
CGGGRIDEANQ

SEQ ID NO: 47 - protein, 11 aa, synthetic construct
  REGION 1..11: note = SNAP-25 antigen
CGGGRIDEANK

SEQ ID NO: 48 - protein, 88 aa, synthetic construct
  REGION 1..88: note = BirA-HisTag(r)-SNAP-25-134-197
MGGGLNDIFEAQKIEWHHHHHHHHIRRVTNDARENEMDENLEQVSGIIGNLRHMALDMGNEIDTQNRQIDRIMEKADSNKTRIDEANQ

SEQ ID NO: 49 - protein, 97 aa, synthetic construct
  REGION 1..97: note = BirA-HisTag(r)-SNAP-25-134-206
MGGGLNDIFEAQKIEWHHHHHHHHIRRVTNDARENEMDENLEQVSGIIGNLRHMALDMGNEIDTQNRQIDRIMEKADSNKTRIDEANQRATKMLGSG

SEQ ID NO: 50 - protein, 16 aa, synthetic construct
  REGION 1..16: note = BirA peptide
GGGLNDIFEAQKIEWH

SEQ ID NO: 51 - DNA, 7570 bp, synthetic construct
  misc_feature 1..7570: note = pQBI-25/GFP-BoNT/A-LC expression construct.
  source 1..7570: mol_type = other DNA
gacggatcgggagatctcccgatcccctatggtcgactctcagtacaatctgctctgatgccgcatagttaagccagtatctgctccctgcttgtgtgttggaggtcgctgagtagtgcgcgagcaaaatttaagctacaacaaggcaaggcttgaccgacaattgcatgaagaatctgcttagggttaggcgttttgcgctgcttcgcctcgaggcctggccattgcatacgttgtatccatatcataatatgtacatttatattggctcatgtccaacattaccgccatgttgacattgattattgactagttattaatagtaatcaattacggggtcattagttcatagcccatatatggagttccgcgttacataacttacggtaaatggcccgcctggctgaccgcccaacgacccccgcccattgacgtcaataatgacgtatgttcccatagtaacgccaatagggactttccattgacgtcaatgggtggagtatttacggtaaactgcccacttggcagtacatcaagtgtatcatatgccaagtacgccccctattgacgtcaatgacggtaaatggcccgcctggcattatgcccagtacatgaccttatgggactttcctacttggcagtacatctacgtattagtcatcgctattaccatggtgatgcggttttggcagtacatcaatgggcgtggatagcggtttgactcacggggatttccaagtctccaccccattgacgtcaatgggagtttgttttggcaccaaaatcaacgggactttccaaaatgtcgtaacaactccgccccattgacgcaaatgggcggtaggcgtgtacggtgggaggtctatataagcagagctcgtttagtgaaccgtcagatcgcctggagacgccatccacgctgttttgacctccatagaagacaccgggaccgatccagcctccgcgggccaccatggagggcccggttaccggtaccggatccagatatctgggcggccgctcagcaagcttcgcgaattcgggaggcggaggtggagctagcaaaggagaagaactcttcactggagttgtcccaattcttgttgaattagatggtgatgttaacggccacaagttctctgtcagtggagagggtgaaggtgatgcaacatacggaaaacttaccctgaagttcatctgcactactggcaaactgcctgttccatggccaacactagtcactactctgtgctatggtgttcaatgcttttcaagatacccggatcatatgaaacggcatgactttttcaagagtgccatgcccgaaggttatgtacaggaaaggaccatcttcttcaaagatgacggcaactacaagacacgtgctgaagtcaagtttgaaggtgatacccttgttaatagaatcgagttaaaaggtattgacttcaaggaagatggcaacattctgggacacaaattggaatacaactataactcacacaatgtatacatcatggcagacaaacaaaagaatggaatcaaagtgaacttcaagacccgccacaacattgaagatggaagcgttcaactagcagaccattatcaacaaaatactccaattggcgatggccctgtccttttaccagacaaccattacctgtccacacaatctgccctttcgaaagatcccaacgaaaagagagaccacatggtccttcttgagtttgtaacagctgctgggattacacatggcatggatgaactgtacaacatcgatggaggcggaggtggaccttttgttaataaacaatttaattataaagatcctgtaaatggtgttgatattgcttatataaaaattccaaatgcaggacaaatgcaaccagtaaaagcttttaaaattcataataaaatatgggttattccagaaagagatacatttacaaatcctgaagaaggagatttaaatccaccaccagaagcaaaacaagttccagtttcatattatgattcaacatatttaagtacagataatgaaaaagataattatttaaagggagttacaaaattatttgagagaatttattcaactgatcttggaagaatgttgttaacatcaatagtaaggggaataccattttggggtggaagtacaatagatacagaattaaaagttattgatactaattgtattaatgtgatacaaccagatggtagttatagatcagaagaacttaatctagtaataataggaccctcagctgatattatacagtttgaatgtaaaagctttggacatgaagttttgaatcttacgcgaaatggttatggctctactcaatacattagatttagcccagattttacatttggttttgaggagtcacttgaagttgatacaaatcctcttttaggtgcaggcaaatttgctacagatccagcagtaacattagcacatgaacttatacatgctggacatagattatatggaatagcaattaatccaaatagggtttttaaagtaaatactaatgcctattatgaaatgagtgggttagaagtaagctttgaggaacttagaacatttgggggacatgatgcaaagtttatagatagtttacaggaaaacgaatttcgtctatattattataataagtttaaagatatagcaagtacacttaataaagctaaatcaatagtaggtactactgcttcattacagtatatgaaaaatgtttttaaagagaaatatctcctatctgaagatacatctggaaaattttcggtagataaattaaaatttgataagttatacaaaatgttaacagagatttacacagaggataattttgttaagttttttaaagtacttaacagaaaaacatatttgaattttgataaagccgtatttaagataaatatagtacctaaggtaaattacacaatatatgatggatttaatttaagaaatacaaatttagcagcaaactttaatggtcaaaatacagaaattaataatatgaattttactaaactaaaaaattttactggattgtttgaattttataagttgctatgtgtaagagggataatcacttcgaaatgaacgcgttggccctattctatagtgtcacctaaatgctagagctcgctgatcagcctcgactgtgccttctagttgccagccatctgttgtttgcccctcccccgtgccttccttgaccctggaaggtgccactcccactgtcctttcctaataaaatgaggaaattgcatcgcattgtctgagtaggtgtcattctattctggggggtggggtggggcaggacagcaagggggaggattgggaagacaatagcaggcatgctggggatgcggtgggctctatggcttctgaggcggaaagaaccagctggggctctagggggtatccccacgcgccctgtagcggcgcattaagcgcggcgggtgtggtggttacgcgcagcgtgaccgctacacttgccagcgccctagcgcccgctcctttcgctttcttcccttcctttctcgccacgttcgccggctttccccgtcaagctctaaatcggggcatccctttagggttccgatttagtgctttacggcacctcgaccccaaaaaacttgattagggtgatggttcacgtagtgggccatcgccctgatagacggtttttcgccctttgacgttggagtccacgttctttaatagtggactcttgttccaaactggaacaacactcaaccctatctcggtctattcttttgatttataagggattttggggatttcggcctattggttaaaaaatgagctgatttaacaaaaatttaacgcgaattaattctgtggaatgtgtgtcagttagggtgtggaaagtccccaggctccccaggcaggcagaagtatgcaaagcatgcatctcaattagtcagcaaccaggtgtggaaagtccccaggctccccagcaggcagaagtatgcaaagcatgcatctcaattagtcagcaaccatagtcccgcccctaactccgcccatcccgcccctaactccgcccagttccgcccattctccgccccatggctgactaattttttttatttatgcagaggccgaggccgcctctgcctctgagctattccagaagtagtgaggaggcttttttggaggcctaggcttttgcaaaaagctcccgggagcttgtatatccattttcggatctgatcaagagacaggatgaggatcgtttcgcatgattgaacaagatggattgcacgcaggttctccggccgcttgggtggagaggctattcggctatgactgggcacaacagacaatcggctgctctgatgccgccgtgttccggctgtcagcgcaggggcgcccggttctttttgtcaagaccgacctgtccggtgccctgaatgaactgcaggacgaggcagcgcggctatcgtggctggccacgacgggcgttccttgcgcagctgtgctcgacgttgtcactgaagcgggaagggactggctgctattgggcgaagtgccggggcaggatctcctgtcatctcaccttgctcctgccgagaaagtatccatcatggctgatgcaatgcggcggctgcatacgcttgatccggctacctgcccattcgaccaccaagcgaaacatcgcatcgagcgagcacgtactcggatggaagccggtcttgtcgatcaggatgatctggacgaagagcatcaggggctcgcgccagccgaactgttcgccaggctcaaggcgcgcatgcccgacggcgaggatctcgtcgtgacccatggcgatgcctgcttgccgaatatcatggtggaaaatggccgcttttctggattcatcgactgtggccggctgggtgtggcggaccgctatcaggacatagcgttggctacccgtgatattgctgaagagcttggcggcgaatgggctgaccgcttcctcgtgctttacggtatcgccgctcccgattcgcagcgcatcgccttctatcgccttcttgacgagttcttctgagcgggactctggggttcgaaatgaccgaccaagcgacgcccaacctgccatcacgagatttcgattccaccgccgccttctatgaaaggttgggcttcggaatcgttttccgggacgccggctggatgatcctccagcgcggggatctcatgctggagttcttcgcccaccccaacttgtttattgcagcttataatggttacaaataaagcaatagcatcacaaatttcacaaataaagcatttttttcactgcattctagttgtggtttgtccaaactcatcaatgtatcttatcatgtctgtataccgtcgacctctagctagagcttggcgtaatcatggtcatagctgtttcctgtgtgaaattgttatccgctcacaattccacacaacatacgagccggaagcataaagtgtaaagcctggggtgcctaatgagtgagctaactcacattaattgcgttgcgctcactgcccgctttccagtcgggaaacctgtcgtgccagctgcattaatgaatcggccaacgcgcggggagaggcggtttgcgtattgggcgctcttccgcttcctcgctcactgactcgctgcgctcggtcgttcggctgcggcgagcggtatcagctcactcaaaggcggtaatacggttatccacagaatcaggggataacgcaggaaagaacatgtgagcaaaaggccagcaaaaggccaggaaccgtaaaaaggccgcgttgctggcgtttttccataggctccgcccccctgacgagcatcacaaaaatcgacgctcaagtcagaggtggcgaaacccgacaggactataaagataccaggcgtttccccctggaagctccctcgtgcgctctcctgttccgaccctgccgcttaccggatacctgtccgcctttctcccttcgggaagcgtggcgctttctcaatgctcacgctgtaggtatctcagttcggtgtaggtcgttcgctccaagctgggctgtgtgcacgaaccccccgttcagcccgaccgctgcgccttatccggtaactatcgtcttgagtccaacccggtaagacacgacttatcgccactggcagcagccactggtaacaggattagcagagcgaggtatgtaggcggtgctacagagttcttgaagtggtggcctaactacggctacactagaaggacagtatttggtatctgcgctctgctgaagccagttaccttcggaaaaagagttggtagctcttgatccggcaaacaaaccaccgctggtagcggtggtttttttgtttgcaagcagcagattacgcgcagaaaaaaaggatctcaagaagatcctttgatcttttctacggggtctgacgctcagtggaacgaaaactcacgttaagggattttggtcatgagattatcaaaaaggatcttcacctagatccttttaaattaaaaatgaagttttaaatcaatctaaagtatatatgagtaaacttggtctgacagttaccaatgcttaatcagtgaggcacctatctcagcgatctgtctatttcgttcatccatagttgcctgactccccgtcgtgtagataactacgatacgggagggcttaccatctggccccagtgctgcaatgataccgcgagacccacgctcaccggctccagatttatcagcaataaaccagccagccggaagggccgagcgcagaagtggtcctgcaactttatccgcctccatccagtctattaattgttgccgggaagctagagtaagtagttcgccagttaatagtttgcgcaacgttgttgccattgctacaggcatcgtggtgtcacgctcgtcgtttggtatggcttcattcagctccggttcccaacgatcaaggcgagttacatgatcccccatgttgtgcaaaaaagcggttagctccttcggtcctccgatcgttgtcagaagtaagttggccgcagtgttatcactcatggttatggcagcactgcataattctcttactgtcatgccatccgtaagatgcttttctgtgactggtgagtactcaaccaagtcattctgagaatagtgtatgcggcgaccgagttgctcttgcccggcgtcaatacgggataataccgcgccacatagcagaactttaaaagtgctcatcattggaaaacgttcttcggggcgaaaactctcaaggatcttaccgctgttgagatccagttcgatgtaacccactcgtgcacccaactgatcttcagcatcttttactttcaccagcgtttctgggtgagcaaaaacaggaaggcaaaatgccgcaaaaaagggaataagggcgacacggaaatgttgaatactcatactcttcctttttcaatattattgaagcatttatcagggttattgtctcatgagcggatacatatttgaatgtatttagaaaaataaacaaataggggttccgcgcacatttccccgaaaagtgccacctgacgtc

SEQ ID NO: 52 - protein, 682 aa, synthetic construct
  REGION 1..682: note = GFP-BoNT/A light chain amino acid sequence.
ASKGEELFTGVVPILVELDGDVNGHKFSVSGEGEGDATYGKLTLKFICTTGKLPVPWPTLVTTLCYGVQCFSRYPDHMKRHDFFKSAMPEGYVQERTIFFKDDGNYKTRAEVKFEGDTLVNRIELKGIDFKEDGNILGHKLEYNYNSHNVYIMADKQKNGIKVNFKTRHNIEDGSVQLADHYQQNTPIGDGPVLLPDNHYLSTQSALSKDPNEKRDHMVLLEFVTAAGITHGMDELYNIDGGGGGPFVNKQFNYKDPVNGVDIAYIKIPNAGQMQPVKAFKIHNKIWVIPERDTFTNPEEGDLNPPPEAKQVPVSYYDSTYLSTDNEKDNYLKGVTKLFERIYSTDLGRMLLTSIVRGIPFWGGSTIDTELKVIDTNCINVIQPDGSYRSEELNLVIIGPSADIIQFECKSFGHEVLNLTRNGYGSTQYIRFSPDFTFGFEESLEVDTNPLLGAGKFATDPAVTLAHELIHAGHRLYGIAINPNRVFKVNTNAYYEMSGLEVSFEELRTFGGHDAKFIDSLQENEFRLYYYNKFKDIASTLNKAKSIVGTTASLQYMKNVFKEKYLLSEDTSGKFSVDKLKFDKLYKMLTEIYTEDNFVKFFKVLNRKTYLNFDKAVFKINIVPKVNYTIYDGFNLRNTNLAANFNGQNTEINNMNFTKLKNFTGLFEFYKLLCVRGIITSK

SEQ ID NO: 53 - DNA, 6259 bp, synthetic construct
  misc_feature 1..6259: note = pQBI-25/GFP expression construct.
  source 1..6259: mol_type = other DNA
gacggatcgggagatctcccgatcccctatggtcgactctcagtacaatctgctctgatgccgcatagttaagccagtatctgctccctgcttgtgtgttggaggtcgctgagtagtgcgcgagcaaaatttaagctacaacaaggcaaggcttgaccgacaattgcatgaagaatctgcttagggttaggcgttttgcgctgcttcgcctcgaggcctggccattgcatacgttgtatccatatcataatatgtacatttatattggctcatgtccaacattaccgccatgttgacattgattattgactagttattaatagtaatcaattacggggtcattagttcatagcccatatatggagttccgcgttacataacttacggtaaatggcccgcctggctgaccgcccaacgacccccgcccattgacgtcaataatgacgtatgttcccatagtaacgccaatagggactttccattgacgtcaatgggtggagtatttacggtaaactgcccacttggcagtacatcaagtgtatcatatgccaagtacgccccctattgacgtcaatgacggtaaatggcccgcctggcattatgcccagtacatgaccttatgggactttcctacttggcagtacatctacgtattagtcatcgctattaccatggtgatgcggttttggcagtacatcaatgggcgtggatagcggtttgactcacggggatttccaagtctccaccccattgacgtcaatgggagtttgttttggcaccaaaatcaacgggactttccaaaatgtcgtaacaactccgccccattgacgcaaatgggcggtaggcgtgtacggtgggaggtctatataagcagagctcgtttagtgaaccgtcagatcgcctggagacgccatccacgctgttttgacctccatagaagacaccgggaccgatccagcctccgcgggccaccatggagggcccggttaccggtaccggatccagatatctgggcggccgctcagcaagcttcgcgaattcgggaggcggaggtggagctagcaaaggagaagaactcttcactggagttgtcccaattcttgttgaattagatggtgatgttaacggccacaagttctctgtcagtggagagggtgaaggtgatgcaacatacggaaaacttaccctgaagttcatctgcactactggcaaactgcctgttccatggccaacactagtcactactctgtgctatggtgttcaatgcttttcaagatacccggatcatatgaaacggcatgactttttcaagagtgccatgcccgaaggttatgtacaggaaaggaccatcttcttcaaagatgacggcaactacaagacacgtgctgaagtcaagtttgaaggtgatacccttgttaatagaatcgagttaaaaggtattgacttcaaggaagatggcaacattctgggacacaaattggaatacaactataactcacacaatgtatacatcatggcagacaaacaaaagaatggaatcaaagtgaacttcaagacccgccacaacattgaagatggaagcgttcaactagcagaccattatcaacaaaatactccaattggcgatggccctgtccttttaccagacaaccattacctgtccacacaatctgccctttcgaaagatcccaacgaaaagagagaccacatggtccttcttgagtttgtaacagctgctgggattacacatggcatggatgaactgtacaacatcgatggaggcggaggtggatgaacgcgttggccctattctatagtgtcacctaaatgctagagctcgctgatcagcctcgactgtgccttctagttgccagccatctgttgtttgcccctcccccgtgccttccttgaccctggaaggtgccactcccactgtcctttcctaataaaatgaggaaattgcatcgcattgtctgagtaggtgtcattctattctggggggtggggtggggcaggacagcaagggggaggattgggaagacaatagcaggcatgctggggatgcggtgggctctatggcttctgaggcggaaagaaccagctggggctctagggggtatccccacgcgccctgtagcggcgcattaagcgcggcgggtgtggtggttacgcgcagcgtgaccgctacacttgccagcgccctagcgcccgctcctttcgctttcttcccttcctttctcgccacgttcgccggctttccccgtcaagctctaaatcggggcatccctttagggttccgatttagtgctttacggcacctcgaccccaaaaaacttgattagggtgatggttcacgtagtgggccatcgccctgatagacggtttttcgccctttgacgttggagtccacgttctttaatagtggactcttgttccaaactggaacaacactcaaccctatctcggtctattcttttgatttataagggattttggggatttcggcctattggttaaaaaatgagctgatttaacaaaaatttaacgcgaattaattctgtggaatgtgtgtcagttagggtgtggaaagtccccaggctccccaggcaggcagaagtatgcaaagcatgcatctcaattagtcagcaaccaggtgtggaaagtccccaggctccccagcaggcagaagtatgcaaagcatgcatctcaattagtcagcaaccatagtcccgcccctaactccgcccatcccgcccctaactccgcccagttccgcccattctccgccccatggctgactaattttttttatttatgcagaggccgaggccgcctctgcctctgagctattccagaagtagtgaggaggcttttttggaggcctaggcttttgcaaaaagctcccgggagcttgtatatccattttcggatctgatcaagagacaggatgaggatcgtttcgcatgattgaacaagatggattgcacgcaggttctccggccgcttgggtggagaggctattcggctatgactgggcacaacagacaatcggctgctctgatgccgccgtgttccggctgtcagcgcaggggcgcccggttctttttgtcaagaccgacctgtccggtgccctgaatgaactgcaggacgaggcagcgcggctatcgtggctggccacgacgggcgttccttgcgcagctgtgctcgacgttgtcactgaagcgggaagggactggctgctattgggcgaagtgccggggcaggatctcctgtcatctcaccttgctcctgccgagaaagtatccatcatggctgatgcaatgcggcggctgcatacgcttgatccggctacctgcccattcgaccaccaagcgaaacatcgcatcgagcgagcacgtactcggatggaagccggtcttgtcgatcaggatgatctggacgaagagcatcaggggctcgcgccagccgaactgttcgccaggctcaaggcgcgcatgcccgacggcgaggatctcgtcgtgacccatggcgatgcctgcttgccgaatatcatggtggaaaatggccgcttttctggattcatcgactgtggccggctgggtgtggcggaccgctatcaggacatagcgttggctacccgtgatattgctgaagagcttggcggcgaatgggctgaccgcttcctcgtgctttacggtatcgccgctcccgattcgcagcgcatcgccttctatcgccttcttgacgagttcttctgagcgggactctggggttcgaaatgaccgaccaagcgacgcccaacctgccatcacgagatttcgattccaccgccgccttctatgaaaggttgggcttcggaatcgttttccgggacgccggctggatgatcctccagcgcggggatctcatgctggagttcttcgcccaccccaacttgtttattgcagcttataatggttacaaataaagcaatagcatcacaaatttcacaaataaagcatttttttcactgcattctagttgtggtttgtccaaactcatcaatgtatcttatcatgtctgtataccgtcgacctctagctagagcttggcgtaatcatggtcatagctgtttcctgtgtgaaattgttatccgctcacaattccacacaacatacgagccggaagcataaagtgtaaagcctggggtgcctaatgagtgagctaactcacattaattgcgttgcgctcactgcccgctttccagtcgggaaacctgtcgtgccagctgcattaatgaatcggccaacgcgcggggagaggcggtttgcgtattgggcgctcttccgcttcctcgctcactgactcgctgcgctcggtcgttcggctgcggcgagcggtatcagctcactcaaaggcggtaatacggttatccacagaatcaggggataacgcaggaaagaacatgtgagcaaaaggccagcaaaaggccaggaaccgtaaaaaggccgcgttgctggcgtttttccataggctccgcccccctgacgagcatcacaaaaatcgacgctcaagtcagaggtggcgaaacccgacaggactataaagataccaggcgtttccccctggaagctccctcgtgcgctctcctgttccgaccctgccgcttaccggatacctgtccgcctttctcccttcgggaagcgtggcgctttctcaatgctcacgctgtaggtatctcagttcggtgtaggtcgttcgctccaagctgggctgtgtgcacgaaccccccgttcagcccgaccgctgcgccttatccggtaactatcgtcttgagtccaacccggtaagacacgacttatcgccactggcagcagccactggtaacaggattagcagagcgaggtatgtaggcggtgctacagagttcttgaagtggtggcctaactacggctacactagaaggacagtatttggtatctgcgctctgctgaagccagttaccttcggaaaaagagttggtagctcttgatccggcaaacaaaccaccgctggtagcggtggtttttttgtttgcaagcagcagattacgcgcagaaaaaaaggatctcaagaagatcctttgatcttttctacggggtctgacgctcagtggaacgaaaactcacgttaagggattttggtcatgagattatcaaaaaggatcttcacctagatccttttaaattaaaaatgaagttttaaatcaatctaaagtatatatgagtaaacttggtctgacagttaccaatgcttaatcagtgaggcacctatctcagcgatctgtctatttcgttcatccatagttgcctgactccccgtcgtgtagataactacgatacgggagggcttaccatctggccccagtgctgcaatgataccgcgagacccacgctcaccggctccagatttatcagcaataaaccagccagccggaagggccgagcgcagaagtggtcctgcaactttatccgcctccatccagtctattaattgttgccgggaagctagagtaagtagttcgccagttaatagtttgcgcaacgttgttgccattgctacaggcatcgtggtgtcacgctcgtcgtttggtatggcttcattcagctccggttcccaacgatcaaggcgagttacatgatcccccatgttgtgcaaaaaagcggttagctccttcggtcctccgatcgttgtcagaagtaagttggccgcagtgttatcactcatggttatggcagcactgcataattctcttactgtcatgccatccgtaagatgcttttctgtgactggtgagtactcaaccaagtcattctgagaatagtgtatgcggcgaccgagttgctcttgcccggcgtcaatacgggataataccgcgccacatagcagaactttaaaagtgctcatcattggaaaacgttcttcggggcgaaaactctcaaggatcttaccgctgttgagatccagttcgatgtaacccactcgtgcacccaactgatcttcagcatcttttactttcaccagcgtttctgggtgagcaaaaacaggaaggcaaaatgccgcaaaaaagggaataagggcgacacggaaatgttgaatactcatactcttcctttttcaatattattgaagcatttatcagggttattgtctcatgagcggatacatatttgaatgtatttagaaaaataaacaaataggggttccgcgcacatttccccgaaaagtgccacctgacgtc

SEQ ID NO: 54 - protein, 245 aa, synthetic construct
  REGION 1..245: note = GFP amino acid sequence.
ASKGEELFTGVVPILVELDGDVNGHKFSVSGEGEGDATYGKLTLKFICTTGKLPVPWPTLVTTLCYGVQCFSRYPDHMKRHDFFKSAMPEGYVQERTIFFKDDGNYKTRAEVKFEGDTLVNRIELKGIDFKEDGNILGHKLEYNYNSHNVYIMADKQKNGIKVNFKTRHNIEDGSVQLADHYQQNTPIGDGPVLLPDNHYLSTQSALSKDPNEKRDHMVLLEFVTAAGITHGMDELYNIDGGGGG

SEQ ID NO: 55 - protein, 4 aa, synthetic construct
  REGION 1..4: note = G-spacer flexible spacer
GGGG

SEQ ID NO: 56 - protein, 5 aa, synthetic construct
  REGION 1..5: note = G-spacer flexible spacer
GGGGS

SEQ ID NO: 57 - protein, 4 aa, synthetic construct
  REGION 1..4: note = A-spacer flexible spacer
AAAA

SEQ ID NO: 58 - protein, 5 aa, synthetic construct
  REGION 1..5: note = A-spacer flexible spacer
AAAAV

SEQ ID NO: 59 - protein, 821 aa, Homo sapiens
MVSWGRFICLVVVTMATLSLARPSFSLVEDTTLEPEEPPTKYQISQPEVYVAAPGESLEVRCLLKDAAVISWTKDGVHLGPNNRTVLIGEYLQIKGATPRDSGLYACTASRTVDSETWYFMVNVTDAISSGDDEDDTDGAEDFVSENSNNKRAPYWTNTEKMEKRLHAVPAANTVKFRCPAGGNPMPTMRWLKNGKEFKQEHRIGGYKVRNQHWSLIMESVVPSDKGNYTCVVENEYGSINHTYHLDVVERSPHRPILQAGLPANASTVVGGDVEFVCKVYSDAQPHIQWIKHVEKNGSKYGPDGLPYLKVLKAAGVNTTDKEIEVLYIRNVTFEDAGEYTCLAGNSIGISFHSAWLTVLPAPGREKEITASPDYLEIAIYCIGVFLIACMVVTVILCRMKNTTKKPDFSSQPAVHKLTKRIPLRRQVTVSAESSSSMNSNTPLVRITTRLSSTADTPMLAGVSEYELPEDPKWEFPRDKLTLGKPLGEGCFGQVVMAEAVGIDKDKPKEAVTVAVKMLKDDATEKDLSDLVSEMEMMKMIGKHKNIINLLGACTQDGPLYVIVEYASKGNLREYLRARRPPGMEYSYDINRVPEEQMTFKDLVSCTYQLARGMEYLASQKCIHRDLAARNVLVTENNVMKIADFGLARDINNIDYYKKTTNGRLPVKWMAPEALFDRVYTHQSDVWSFGVLMWEIFTLGGSPYPGIPVEELFKLLKEGHRMDKPANCTNELYMMMRDCWHAVPSQRPTFKQLVEDLDRILTLTTNEEYLDLSQPLEQYSPSYPDTRSSCSSGDDSVFSPDPMPYEPCLPQYPHINGSVKT

SEQ ID NO: 60 - protein, 822 aa, Homo sapiens
MVSWGRFICLVVVTMATLSLARPSFSLVEDTTLEPEEPPTKYQISQPEVYVAAPGESLEVRCLLKDAAVISWTKDGVHLGPNNRTVLIGEYLQIKGATPRDSGLYACTASRTVDSETWYFMVNVTDAISSGDDEDDTDGAEDFVSENSNNKRAPYWTNTEKMEKRLHAVPAANTVKFRCPAGGNPMPTMRWLKNGKEFKQEHRIGGYKVRNQHWSLIMESVVPSDKGNYTCVVENEYGSINHTYHLDVVERSPHRPILQAGLPANASTVVGGDVEFVCKVYSDAQPHIQWIKHVEKNGSKYGPDGLPYLKVLKHSGINSSNAEVLALFNVTEADAGEYICKVSNYIGQANQSAWLTVLPKQQAPGREKEITASPDYLEIAIYCIGVFLIACMVVTVILCRMKNTTKKPDFSSQPAVHKLTKRIPLRRQVTVSAESSSSMNSNTPLVRITTRLSSTADTPMLAGVSEYELPEDPKWEFPRDKLTLGKPLGEGCFGQVVMAEAVGIDKDKPKEAVTVAVKMLKDDATEKDLSDLVSEMEMMKMIGKHKNIINLLGACTQDGPLYVIVEYASKGNLREYLRARRPPGMEYSYDINRVPEEQMTFKDLVSCTYQLARGMEYLASQKCIHRDLAARNVLVTENNVMKIADFGLARDINNIDYYKKTTNGRLPVKWMAPEALFDRVYTHQSDVWSFGVLMWEIFTLGGSPYPGIPVEELFKLLKEGHRMDKPANCTNELYMMMRDCWHAVPSQRPTFKQLVEDLDRILTLTTNEEYLDLSQPLEQYSPSYPDTRSSCSSGDDSVFSPDPMPYEPCLPQYPHINGSVKT

SEQ ID NO: 61 - protein, 769 aa, Homo sapiens
MVSWGRFICLVVVTMATLSLARPSFSLVEDTTLEPEEPPTKYQISQPEVYVAAPGESLEVRCLLKDAAVISWTKDGVHLGPNNRTVLIGEYLQIKGATPRDSGLYACTASRTVDSETWYFMVNVTDAISSGDDEDDTDGAEDFVSENSNNKRAPYWTNTEKMEKRLHAVPAANTVKFRCPAGGNPMPTMRWLKNGKEFKQEHRIGGYKVRNQHWSLIMESVVPSDKGNYTCVVENEYGSINHTYHLDVVERSPHRPILQAGLPANASTVVGGDVEFVCKVYSDAQPHIQWIKHVEKNGSKYGPDGLPYLKVLKHSGINSSNAEVLALFNVTEADAGEYICKVSNYIGQANQSAWLTVLPKQQAPGREKEITASPDYLEIAIYCIGVFLIACMVVTVILCRMKNTTKKPDFSSQPAVHKLTKRIPLRRQVTVSAESSSSMNSNTPLVRITTRLSSTADTPMLAGVSEYELPEDPKWEFPRDKLTLGKPLGEGCFGQVVMAEAVGIDKDKPKEAVTVAVKMLKDDATEKDLSDLVSEMEMMKMIGKHKNIINLLGACTQDGPLYVIVEYASKGNLREYLRARRPPGMEYSYDINRVPEEQMTFKDLVSCTYQLARGMEYLASQKCIHRDLAARNVLVTENNVMKIADFGLARDINNIDYYKKTTNGRLPVKWMAPEALFDRVYTHQSDVWSFGVLMWEIFTLGGSPYPGIPVEELFKLLKEGHRMDKPANCTNELYMMMRDCWHAVPSQRPTFKQLVEDLDRILTLTTNEI

SEQ ID NO: 62 - protein, 709 aa, Homo sapiens
MVSWGRFICLVVVTMATLSLARPSFSLVEDTTLEPEEPPTKYQISQPEVYVAAPGESLEVRCLLKDAAVISWTKDGVHLGPNNRTVLIGEYLQIKGATPRDSGLYACTASRTVDSETWYFMVNVTDAISSGDDEDDTDGAEDFVSENSNNKRAPYWTNTEKMEKRLHAVPAANTVKFRCPAGGNPMPTMRWLKNGKEFKQEHRIGGYKVRNQHWSLIMESVVPSDKGNYTCVVENEYGSINHTYHLDVVAPGREKEITASPDYLEIAIYCIGVFLIACMVVTVILCRMKNTTKKPDFSSQPAVHKLTKRIPLRRQVTVSAESSSSMNSNTPLVRITTRLSSTADTPMLAGVSEYELPEDPKWEFPRDKLTLGKPLGEGCFGQVVMAEAVGIDKDKPKEAVTVAVKMLKDDATEKDLSDLVSEMEMMKMIGKHKNIINLLGACTQDGPLYVIVEYASKGNLREYLRARRPPGMEYSYDINRVPEEQMTFKDLVSCTYQLARGMEYLASQKCIHRDLAARNVLVTENNVMKIADFGLARDINNIDYYKKTTNGRLPVKWMAPEALFDRVYTHQSDVWSFGVLMWEIFTLGGSPYPGIPVEELFKLLKEGHRMDKPANCTNELYMMMRDCWHAVPSQRPTFKQLVEDLDRILTLTTNEEYLDLSQPLEQYSPSYPDTRSSCSSGDDSVFSPDPMPYEPCLPQYPHINGSVKT

SEQ ID NO: 63 - protein, 707 aa, Homo sapiens
MVSWGRFICLVVVTMATLSLARPSFSLVEDTTLEPEDAISSGDDEDDTDGAEDFVSENSNNKRAPYWTNTEKMEKRLHAVPAANTVKFRCPAGGNPMPTMRWLKNGKEFKQEHRIGGYKVRNQHWSLIMESVVPSDKGNYTCVVENEYGSINHTYHLDVVERSPHRPILQAGLPANASTVVGGDVEFVCKVYSDAQPHIQWIKHVEKNGSKYGPDGLPYLKVLKAAGVNTTDKEIEVLYIRNVTFEDAGEYTCLAGNSIGISFHSAWLTVLPAPGREKEITASPDYLEIAIYCIGVFLIACMVVTVILCRMKNTTKKPDFSSQPAVHKLTKRIPLRRQVTVSAESSSSMNSNTPLVRITTRLSSTADTPMLAGVSEYELPEDPKWEFPRDKLTLGKPLGEGCFGQVVMAEAVGIDKDKPKEAVTVAVKMLKDDATEKDLSDLVSEMEMMKMIGKHKNIINLLGACTQDGPLYVIVEYASKGNLREYLRARRPPGMEYSYDINRVPEEQMTFKDLVSCTYQLARGMEYLASQKCIHRDLAARNVLVTENNVMKIADFGLARDINNIDYYKKTTNGRLPVKWMAPEALFDRVYTHQSDVWSFGVLMWEIFTLGGSPYPGIPVEELFKLLKEGHRMDKPANCTNELYMMMRDCWHAVPSQRPTFKQLVEDLDRILTLTTNEEEKKVSGAVDCHKPPCNPSHLPCVLAVDQ

SEQ ID NO: 64 - protein, 706 aa, Homo sapiens
MVSWGRFICLVVVTMATLSLARPSFSLVEDTTLEPEGAPYWTNTEKMEKRLHAVPAANTVKFRCPAGGNPMPTMRWLKNGKEFKQEHRIGGYKVRNQHWSLIMESVVPSDKGNYTCVVENEYGSINHTYHLDVVERSPHRPILQAGLPANASTVVGGDVEFVCKVYSDAQPHIQWIKHVEKNGSKYGPDGLPYLKVLKAAGVNTTDKEIEVLYIRNVTFEDAGEYTCLAGNSIGISFHSAWLTVLPAPGREKEITASPDYLEIAIYCIGVFLIACMVVTVILCRMKNTTKKPDFSSQPAVHKLTKRIPLRRQVTVSAESSSSMNSNTPLVRITTRLSSTADTPMLAGVSEYELPEDPKWEFPRDKLTLGKPLGEGCFGQVVMAEAVGIDKDKPKEAVTVAVKMLKDDATEKDLSDLVSEMEMMKMIGKHKNIINLLGACTQDGPLYVIVEYASKGNLREYLRARRPPGMEYSYDINRVPEEQMTFKDLVSCTYQLARGMEYLASQKCIHRDLAARNVLVTENNVMKIADFGLARDINNIDYYKKTTNGRLPVKWMAPEALFDRVYTHQSDVWSFGVLMWEIFTLGGSPYPGIPVEELFKLLKEGHRMDKPANCTNELYMMMRDCWHAVPSQRPTFKQLVEDLDRILTLTTNEEYLDLSQPLEQYSPSYPDTRSSCSSGDDSVFSPDPMPYEPCLPQYPHINGSVKT

SEQ ID NO: 65 - protein, 705 aa, Homo sapiens
MVSWGRFICLVVVTMATLSLARPSFSLVEDTTLEPEEPPTKYQISQPEVYVAAPGESLEVRCLLKDAAVISWTKDGVHLGPNNRTVLIGEYLQIKGATPRDSGLYACTASRTVDSETWYFMVNVTDAISSGDDEDDTDGAEDFVSENSNNKRAPYWTNTEKMEKRLHAVPAANTVKFRCPAGGNPMPTMRWLKNGKEFKQEHRIGGYKVRNQHWSLIMESVVPSDKGNYTCVVENEYGSINHTYHLDVVERSPHRPILQAGLPANASTVVGGDVEFVCKVYSDAQPHIQWIKHVEKNGSKYGPDGLPYLKVLKVSAESSSSMNSNTPLVRITTRLSSTADTPMLAGVSEYELPEDPKWEFPRDKLTLGKPLGEGCFGQVVMAEAVGIDKDKPKEAVTVAVKMLKDDATEKDLSDLVSEMEMMKMIGKHKNIINLLGACTQDGPLYVIVEYASKGNLREYLRARRPPGMEYSYDINRVPEEQMTFKDLVSCTYQLARGMEYLASQKCIHRDLAARNVLVTENNVMKIADFGLARDINNIDYYKKTTNGRLPVKWMAPEALFDRVYTHQSDVWSFGVLMWEIFTLGGSPYPGIPVEELFKLLKEGHRMDKPANCTNELYMMMRDCWHAVPSQRPTFKQLVEDLDRILTLTTNEEYLDLSQPLEQYSPSYPDTRSSCSSGDDSVFSPDPMPYEPCLPQYPHINGSVKT

SEQ ID NO: 66 - protein, 704 aa, Homo sapiens
MVSWGRFICLVVVTMATLSLARPSFSLVEDTTLEPEGAPYWTNTEKMEKRLHAVPAANTVKFRCPAGGNPMPTMRWLKNGKEFKQEHRIGGYKVRNQHWSLIMESVVPSDKGNYTCVVENEYGSINHTYHLDVVERSPHRPILQAGLPANASTVVGGDVEFVCKVYSDAQPHIQWIKHVEKNGSKYGPDGLPYLKVLKAAGVNTTDKEIEVLYIRNVTFEDAGEYTCLAGNSIGISFHSAWLTVLPAPGREKEITASPDYLEIAIYCIGVFLIACMVVTVILCRMKNTTKKPDFSSQPAVHKLTKRIPLRRQVSAESSSSMNSNTPLVRITTRLSSTADTPMLAGVSEYELPEDPKWEFPRDKLTLGKPLGEGCFGQVVMAEAVGIDKDKPKEAVTVAVKMLKDDATEKDLSDLVSEMEMMKMIGKHKNIINLLGACTQDGPLYVIVEYASKGNLREYLRARRPPGMEYSYDINRVPEEQMTFKDLVSCTYQLARGMEYLASQKCIHRDLAARNVLVTENNVMKIADFGLARDINNIDYYKKTTNGRLPVKWMAPEALFDRVYTHQSDVWSFGVLMWEIFTLGGSPYPGIPVEELFKLLKEGHRMDKPANCTNELYMMMRDCWHAVPSQRPTFKQLVEDLDRILTLTTNEEYLDLSQPLEQYSPSYPDTRSSCSSGDDSVFSPDPMPYEPCLPQYPHINGSVKT

SEQ ID NO: 67 - protein, 680 aa, Homo sapiens
MVSWGRFICLVVVTMATLSLARPSFSLVEDTTLEPEDAISSGDDEDDTDGAEDFVSENSNNKRAPYWTNTEKMEKRLHAVPAANTVKFRCPAGGNPMPTMRWLKNGKEFKQEHRIGGYKVRNQHWSLIMESVVPSDKGNYTCVVENEYGSINHTYHLDVVERSPHRPILQAGLPANASTVVGGDVEFVCKVYSDAQPHIQWIKHVEKNGSKYGPDGLPYLKVLKHSGINSSNAEVLALFNVTEADAGEYICKVSNYIGQANQSAWLTVLPKQQAPGREKEITASPDYLEIAIYCIGVFLIACMVVTVILCRMKNTTKKPDFSSQPAVHKLTKRIPLRRQVTVSAESSSSMNSNTPLVRITTRLSSTADTPMLAGVSEYELPEDPKWEFPRDKLTLGKPLGEGCFGQVVMAEAVGIDKDKPKEAVTVAVKMLKDDATEKDLSDLVSEMEMMKMIGKHKNIINLLGACTQDGPLYVIVEYASKGNLREYLRARRPPGMEYSYDINRVPEEQMTFKDLVSCTYQLARGMEYLASQKCIHRDLAARNVLVTENNVMKIADFGLARDINNIDYYKKTTNGRLPVKWMAPEALFDRVYTHQSDVWSFGVLMWEIFTLGGSPYPGIPVEELFKLLKEGHRMDKPANCTNELYMMMRDCWHAVPSQRPTFKQLVEDLDRILTLTTNEI

SEQ ID NO: 68 - protein, 396 aa, Homo sapiens [sequence omitted]

SEQ ID NO: 69 - protein, 317 aa, Homo sapiens
MVSWGRFICLVVVTMATLSLARPSFSLVEDTTLEPEEPPTKYQISQPEVYVAAPGESLEVRCLLKDAAVISWTKDGVHLGPNNRTVLIGEYLQIKGATPRDSGLYACTASRTVDSETWYFMVNVTDAISSGDDEDDTDGAEDFVSENSNNKRAPYWTNTEKMEKRLHAVPAANTVKFRCPAGGNPMPTMRWLKNGKEFKQEHRIGGYKVRNQHWSLIMESVVPSDKGNYTCVVENEYGSINHTYHLDVVERSPHRPILQAGLPANASTVVGGDVEFVCKVYSDAQPHIQWIKHVEKNGSKYGPDGLPYLKVLKVRTF

SEQ ID NO: 70 - protein, 266 aa, Homo sapiens [sequence omitted]

SEQ ID NO: 71 - DNA, 336 bp, Mus musculus
  source 1..336: mol_type = other DNA
caggtgaagctgcaggagtctggcgctgagttggtgaaacctggggcttcagtgaagatatcctgcaaggcttctggctacatcttcactgaccatgctcttcactgggtgaggcagaagcctgaacagggcctggaatggattgggtatatttttcccggaaatggtaatattgagtacaatgagaagttcaagggcaaggccacactgactgcagacaaatcctccagtactgcctacatgcagctcaacagcctgacatctggagattctgcaatgtatttctgtaaaaagatggactactggggccaagggaccacggtcaccgtctcctca

SEQ ID NO: 72 - protein, 111 aa, Mus musculus
VKLQESGAELVKPGASVKISCKASGYIFTDHALHWVRQKPEQGLEWIGYIFPGNGNIEYNEKFKGKATLTADKSSSTAYMQLNSLTSGDSAMYFCKKMDYWGQGTTVTVSS

SEQ ID NO: 73 - DNA, 336 bp, Mus musculus
  source 1..336: mol_type = other DNA
caggtgaagctgcaggagtctggcgctgagttggtgaaacctggggcttcagtgaagatctcctgcaaggcttctggttacaccttcactgaccattctattcactgggtgaagcagaagcctggacagggcctagaatggattggatatctttttcccggaaatggtaattttgaatataatgagaaattcaagggcaaggccacactgactgcagacaaatcctccagcactgcctacatgcacctcaacagcctgacatctgaggattctgcagtgtatttctgtaaaaagatggactactggggccaagggaccacggtcaccgtctcctca

SEQ ID NO: 74 - protein, 111 aa, Mus musculus
VKLQESGAELVKPGASVKISCKASGYTFTDHSIHWVKQKPGQGLEWIGYLFPGNGNFEYNEKFKGKATLTADKSSSTAYMHLNSLTSEDSAVYFCKKMDYWGQGTTVTVSS

SEQ ID NO: 75 - DNA, 336 bp, Mus musculus
  source 1..336: mol_type = other DNA
caggttcagctgcagcagtccgacgctgagttggtgaaacctggggcttcagtgaagatatcctgcagggcttctggctacaccttcactgaccattctattcactgggtgaagcagcagcctggccagggcctggaatggatcggatatatttttcccggaaatggaaatattgaatacaatgacaaattcaagggcaaggccacactgactgcagacaaatcctccggcactgcctacatgcagctcaacagcctgacatctgaggattctgcagtgtatttctgtaaaaggatggggtactggggtcaaggaacctcagtcaccgtctcctca

SEQ ID NO: 76 - protein, 111 aa, Mus musculus
VQLQQSDAELVKPGASVKISCRASGYTFTDHSIHWVKQQPGQGLEWIGYIFPGNGNIEYNDKFKGKATLTADKSSGTAYMQLNSLTSEDSAVYFCKRMGYWGQGTSVTVSS

SEQ ID NO: 77 - DNA, 360 bp, Mus musculus
  source 1..360: mol_type = other DNA
caggtcaagctgcaggagtctggacctgaactggtaaagcctggggcttcagtgaagatgtcctgcaaggcttctggatacacattcactaactatgttatacactgggtgaagcaaaagcctgggcagggccttgagtggattggatatattaatccttacaatgatggctctaagtacaatgagaagttcaaaggcaaggcctcactgacttcagacaaatcctccagcacagcctacatggagctcagcagcctgacctctgaggactctgcggtctattactgtgcaagacatctcgctaatacctactactactttgactactggggccaagggaccacggtcaccgtctcctca

SEQ ID NO: 78 - protein, 119 aa, Mus musculus
VKLQESGPELVKPGASVKMSCKASGYTFTNYVIHWVKQKPGQGLEWIGYINPYNDGSKYNEKFKGKASLTSDKSSSTAYMELSSLTSEDSAVYYCARHLANTYYYFDYWGQGTTVTVSS

SEQ ID NO: 79 - DNA, 336 bp, Mus musculus
  source 1..336: mol_type = other DNA
caggtcaagctgcaggagtctggcgctgagttggtgaaacctggggcttcagtgaagatctcctgcaaggcttctggctacaccttcactgaccattctattcactgggtgaagcagaagcctggacagggcctagaatggattggatatctttttcccggaaatggtaattttgagtacaatgaaaaattcaagggcaaggccacactgactgcagacaaatcctccagcactgtctacatgtacctcaacagcctgacatctgaggattctgcagtgtatttctgtaaaaggatggggtactggggccaagggaccacggtcaccgtctcctca

SEQ ID NO: 80 - protein, 111 aa, Mus musculus
VKLQESGAELVKPGASVKISCKASGYTFTDHSIHWVKQKPGQGLEWIGYLFPGNGNFEYNEKFKGKATLTADKSSSTVYMYLNSLTSEDSAVYFCKRMGYWGQGTTVTVSS

SEQ ID NO: 81 - DNA, 357 bp, Mus musculus
  source 1..357: mol_type = other DNA
gtgaagctgcaggagtctggacctgaactggtaaagcctggggcttcagtgaagatgtcctgcaaggcttctggatacacattcactaactatgttatacactgggtgaagcaaaagcctgggcagggccttgagtggattggatatattaatccttacaatgatggctctaagtacaatgagaagttcaaaggcaaggcctcactgacttcagacaaatcctccagcacagcctacatggagctcagcagcctgacctctgaggactctgcggtctattactgtgcaagacatctcgctaatacctactactactttgactactggggccaaggcaccactctcacagtctcctca

SEQ ID NO: 82 - protein, 120 aa, Mus musculus
QVQLQESGPELVKPGASVKMSCKASGYTFTNYVIHWVKQKPGQGLEWIGYINPYNDGSKYNEKFKGKASLTSDKSSSTAYMELSSLTSEDSAVYYCARHLANTYYYFDYWGQGTTLTVSS

SEQ ID NO: 83 - DNA, 342 bp, Mus musculus
  source 1..342: mol_type = other DNA
gatgttttgatgacccaaactccactctccctgcctgtcagtcttggagatcaagcctccatctcttgcagatctagtcagagcattgtacatagtaatggaaacacctatttagaatggtacctgcagaaaccaggccagtctccaaagctcctgatctacaaagtttccaaccgattttctggggtcccagacaggttcagtggcagtggatcagggacagatttcacactcaagatcagcagagtggaggctgaggatctgggagtttattactgctttcaaggttcacatgttcctcctacgttcggtgctgggaccaagctggagctgaaacgggct

SEQ ID NO: 84 - protein, 113 aa, Mus musculus
DVLMTQTPLSLPVSLGDQASISCRSSQSIVHSNGNTYLEWYLQKPGQSPKLLIYKVSNRFSGVPDRFSGSGSGTDFTLKISRVEAEDLGVYYCFQGSHVPPTFGAGTKLELKR

SEQ ID NO: 85 - DNA, 324 bp, Mus musculus
  source 1..324: mol_type = other DNA
gacatccagatgactcagtctccagcctccctatctgcatctgtgggagaaactgtcaccatcacatgtcgaacaactgaaaatatttacagttattttgtatggtctcagcagagacagggaaaatctcctcagctccgggtctataatgcaaaatccttagcagaaggtgtgccatcaagtttcaatgtcagtgtatcaggcacacagttttctctgaagatcaatagcctgcagcctgaagattttgggacttatcactgtcaacaccattatggtactccgtacacgttcggaggggggaccaggctggaaataagacgg

SEQ ID NO: 86 - protein, 108 aa, Mus musculus
DIQMTQSPASLSASVGETVTITCRTTENIYSYFVWSQQRQGKSPQLRVYNAKSLAEGVPSSFNVSVSGTQFSLKINSLQPEDFGTYHCQHHYGTPYTFGGGTRLEIRR

SEQ ID NO: 87 - DNA, 336 bp, Mus musculus
  source 1..336: mol_type = other DNA
gacattgtgctgacacagtctcctgcttccttagctgtatctctggggcagagggccaccatctcgtacagggccagcaaaagtgtcagtacatctggctatagttatatgcactggaaccaacagaaaccaggacagccacccagactcctcatctatcttgtatccaacctagaatctggggtccctgccaggttcagtggcagtgggtctgggacagacttcaccctcaacatccatcctgtggaggaggaggatgctgcaacctattactgtcagcacattagggagcttacacgttcggaggggggcaccaagctggaaatcaaacggaga

SEQ ID NO: 88 - protein, 112 aa, Mus musculus
DIVLTQSPASLAVSLGQRATISYRASKSVSTSGYSYMHWNQQKPGQPPRLLIYLVSNLESGVPARFSGSGSGTDFTLNIHPVEEEDAATYYCQHIRELTRSEGGTKLEIKRR

SEQ ID NO: 89 - DNA, 327 bp, Mus musculus
  source 1..327: mol_type = other DNA
gacatcaagatgacccagtctccatcctccatgtatgcatcgctgggagagagagtcactatcacttgcaaggcgagtcaggacattaaaagctatttaagctggtaccagcagaaaccatggaaatctcctaagaccctgatctattatgcaacaagcttggcagatggggtcccatcaagattcagtggcagtggatctgggcaagattattctctaaccatcagcagcctggagtctgacgatacagcaacttattactgtctacagcatggtgagagcccgtacacgttcggaggggggaccaagctggaaataaaacgggct

SEQ ID NO: 90 - protein, 108 aa, Mus musculus
DIKMTQSPSSMYASLGERVTITCKASQDIKSYLSWYQQKPWKSPKTLIYYATSLADGVPSRFSGSGSGQDYSLTISSLESDDTATYYCLQHGESPFTFGSGTKLEIKR

SEQ ID NO: 91 - DNA, 327 bp, Mus musculus
  source 1..327: mol_type = other DNA
gatgttgtgctaactcagtctcctgccaccctgtctgtgactccaggagatagagtcagtctttcctgcagggccagccaaaatattggcaactacctacactggtatcaacagaaatcacatgagtctccaaggcttctcatcaagtatgcttcccagtccatctctgggatcccctccaggttcagtggcagtggatcagtcacagatttcactctcaatatcaacagtgtggagactgaagattttggaatgtatttctgtcaacagagtgacacctggcctctcacgttcggtgctgggaccaagctggagctgaaacgggct

SEQ ID NO: 92 - protein, 108 aa, Mus musculus
DVVLTQSPATLSVTPGDRVSLSCRASQNIGNYLHWYQQKSHESPRLLIKYASQSISGIPSRFSGSGSVTDFTLNINSVETEDFGMYFCQQSDTWPLTFGAGTKLELKR

SEQ ID NO: 93 - protein, 8 aa, Mus musculus
TFTDHSIH

SEQ ID NO: 94 - protein, 8 aa, Mus musculus
TFTNYVIH

SEQ ID NO: 95 - protein, 8 aa, Mus musculus
IFTDHALH

SEQ ID NO: 96 - protein, 17 aa, Mus musculus
YIFPGNGNIEYNDKFKG

SEQ ID NO: 97 - protein, 17 aa, Mus musculus
YLFPGNGNFEYNEKFKG

SEQ ID NO: 98 - protein, 17 aa, Mus musculus
YINPYNDGSKYNEKFKG

SEQ ID NO: 99 - protein, 17 aa, Mus musculus
YIFPGNGNIEYNEKFKG

SEQ ID NO: 100 - protein, 5 aa, Mus musculus
KRMGY

SEQ ID NO: 101 - protein, 5 aa, Mus musculus
KKMDY

SEQ ID NO: 102 - protein, 13 aa, Mus musculus
ARHLANTYYYFDY

SEQ ID NO: 103 - protein, 16 aa, Mus musculus
RSSQSIVHSNGNTYLE

SEQ ID NO: 104 - protein, 11 aa, Mus musculus
RTTENIYSYFV

SEQ ID NO: 105 - protein, 15 aa, Mus musculus
RASKSVSTSGYSYMH

SEQ ID NO: 106 - protein, 11 aa, Mus musculus
KASQDIKSYLS

SEQ ID NO: 107 - protein, 11 aa, Mus musculus
RASQNIGNYLH

SEQ ID NO: 108 - protein, 7 aa, Mus musculus
KVSNRFS

SEQ ID NO: 109 - protein, 7 aa, Mus musculus
NAKSLAE

SEQ ID NO: 110 - protein, 7 aa, Mus musculus
LVSNLES

SEQ ID NO: 111 - protein, 7 aa, Mus musculus
YATSLAD

SEQ ID NO: 112 - protein, 7 aa, Mus musculus
YASQSIS

SEQ ID NO: 113 - protein, 9 aa, Mus musculus
FQGSHVPPT

SEQ ID NO: 114 - protein, 9 aa, Mus musculus
QHHYGTPYT

SEQ ID NO: 115 - protein, 9 aa, Mus musculus
QHIRELTRS

SEQ ID NO: 116 - protein, 9 aa, Mus musculus
LQHGESPFT

SEQ ID NO: 117 - protein, 9 aa, Mus musculus
QQSDTWPLT

SEQ ID NO: 118 - protein, 5 aa, Mus musculus
DHALH

SEQ ID NO: 119 - protein, 5 aa, Mus musculus
DHSIH

SEQ ID NO: 120 - protein, 5 aa, Mus musculus
NYVIH

SEQ ID NO: 121 - protein, 9 aa, Mus musculus
IFPGNGNIE

SEQ ID NO: 122 - protein, 9 aa, Mus musculus
LFPGNGNFE

SEQ ID NO: 123 - protein, 9 aa, Mus musculus
INPYNDGSK

SEQ ID NO: 124 - protein, 11 aa, Mus musculus
HLANTYYYFDY

SEQ ID NO: 125 - protein, 5 aa, Mus musculus
SNGNT

SEQ ID NO: 126 - protein, 5 aa, Mus musculus
ENIYS

SEQ ID NO: 127 - protein, 5 aa, Mus musculus
TSGYS

SEQ ID NO: 128 - protein, 5 aa, Mus musculus
QDIKS

SEQ ID NO: 129 - protein, 5 aa, Mus musculus
QNIGN

SEQ ID NO: 130 - DNA, 4654 bp, Homo sapiens
  source 1..4654: mol_type = other DNA
ggcggcggctggaggagagcgcggtggagagccgagcgggcgggcggcgggtgcggagcgggcgagggagcgcgcgcggccgccacaaagctcgggcgccgcggggctgcatgcggcgtacctggcccggcgcggcgactgctctccgggctggcgggggccggccgcgagccccgggggccccgaggccgcagcttgcctgcgcgctctgagccttcgcaactcgcgagcaaagtttggtggaggcaacgccaagcctgagtcctttcttcctctcgttccccaaatccgagggcagcccgcgggcgtcatgcccgcgctcctccgcagcctggggtacgcgtgaagcccgggaggcttggcgccggcgaagacccaaggaccactcttctgcgtttggagttgctccccgcaaccccgggctcgtcgctttctccatcccgacccacgcggggcgcggggacaacacaggtcgcggaggagcgttgccattcaagtgactgcagcagcagcggcagcgcctcggttcctgagcccaccgcaggctgaaggcattgcgcgtagtccatgcccgtagaggaagtgtgcagatgggattaacgtccacatggagatatggaagaggaccggggattggtaccgtaaccatggtcagctggggtcgtttcatctgcctggtcgtggtcaccatggcaaccttgtccctggcccggccctccttcagtttagttgaggataccacattagagccagaagagccaccaaccaaataccaaatctctcaaccagaagtgtacgtggctgcgccaggggagtcgctagaggtgcgctgcctgttgaaagatgccgccgtgatcagttggactaaggatggggtgcacttggggcccaacaataggacagtgcttattggggagtacttgcagataaagggcgccacgcctagagactccggcctctatgcttgtactgccagtaggactgtagacagtgaaacttggtacttcatggtgaatgtcacagatgccatctcatccggagatgatgaggatgacaccgatggtgcggaagattttgtcagtgagaacagtaacaacaagagagcaccatactggaccaacacagaaaagatggaaaagcggctccatgctgtgcctgcggccaacactgtcaagtttcgctgcccagccggggggaacccaatgccaaccatgcggtggctgaaaaacgggaaggagtttaagcaggagcatcgcattggaggctacaaggtacgaaaccagcactggagcctcattatggaaagtgtggtcccatctgacaagggaaattatacctgtgtagtggagaatgaatacgggtccatcaatcacacgtaccacctggatgttgtggagcgatcgcctcaccggcccatcctccaagccggactgccggcaaatgcctccacagtggtcggaggagacgtagagtttgtctgcaaggtttacagtgatgcccagccccacatccagtggatcaagcacgtggaaaagaacggcagtaaatacgggcccgacgggctgccctacctcaaggttctcaaggccgccggtgttaacaccacggacaaagagattgaggttctctatattcggaatgtaacttttgaggacgctggggaatatacgtgcttggcgggtaattctattgggatatcctttcactctgcatggttgacagttctgccagcgcctggaagagaaaaggagattacagcttccccagactacctggagatagccatttactgcataggggtcttcttaatcgcctgtatggtggtaacagtcatcctgtgccgaatgaagaacacgaccaagaagccagacttcagcagccagccggctgtgcacaagctgaccaaacgtatccccctgcggagacaggtaacagtttcggctgagtccagctcctccatgaactccaacaccccgctggtgaggataacaacacgcctctcttcaacggcagacacccccatgctggcaggggtctccgagtatgaacttccagaggacccaaaatgggagtttccaagagataagctgacactgggcaagcccctgggagaaggttgctttgggcaagtggtcatggcggaagcagtgggaattgacaaagacaagcccaaggaggcggtcaccgtggccgtgaagatgttgaaagatgatgccacagagaaagacctttctgatctggtgtcagagatggagatgatgaagatgattgggaaacacaagaatatcataaatcttcttggagcctgcacacaggatgggcctctctatgtcatagttgagtatgcctctaaaggcaacctccgagaatacctccgagcccggaggccacccgggatggagtactcctatgacattaaccgtgttcctgaggagcagatgaccttcaaggacttggtgtcatgcacctaccagctggccagaggcatggagtacttggcttcccaaaaatgtattcatcgagatttagcagccagaaatgttttggtaacagaaaacaatgtgatgaaaatagcagactttggactcgccagagatatcaacaatatagactattacaaaaagaccaccaatgggcggcttccagtcaagtggatggctccagaagccctgtttgatagagtatacactcatcagagtgatgtctggtccttcggggtgttaatgtgggagatcttcactttagggggctcgccctacccagggattcccgtggaggaactttttaagctgctgaaggaaggacacagaatggataagccagccaactgcaccaacgaactgtacatgatgatgagggactgttggcatgcagtgccctcccagagaccaacgttcaagcagttggtagaagacttggatcgaattctcactctcacaaccaatgaggaatacttggacctcagccaacctctcgaacagtattcacctagttaccctgacacaagaagttcttgttcttcaggagatgattctgttttttctccagaccccatgccttacgaaccatgccttcctcagtatccacacataaacggcagtgttaaaacatgaatgactgtgtctgcctgtccccaaacaggacagcactgggaacctagctacactgagcagggagaccatgcctcccagagcttgttgtctccacttgtatatatggatcagaggagtaaataattggaaaagtaatcagcatatgtgtaaagatttatacagttgaaaacttgtaatcttccccaggaggagaagaaggtttctggagcagtggactgccacaagccaccatgtaacccctctcacctgccgtgcgtactggctgtggaccagtaggactcaaggtggacgtgcgttctgccttccttgttaattttgtaataattggagaagatttatgtcagcacacacttacagagcacaaatgcagtatataggtgctggatgtatgtaaatatattcaaattatgtataaatatatattatatatttacaaggagttattttttgtattgattttaaatggatgtcccaatgcacctagaaaattggtctctctttttttaatagctatttgctaaatgctgttcttacacataatttcttaattttcaccgagcagaggtggaaaaatacttttgctttcagggaaaatggtataacgttaatttattaataaattggtaatatacaaaacaattaatcatttatagttttttttgtaatttaagtggcatttctatgcaggcagcacagcagactagttaatctattgcttggacttaactagttatcagatcctttgaaaagagaatatttacaatatatgactaatttggggaaaatgaagttttgatttatttgtgtttaaatgctgctgtcagacgattgttcttagacctcctaaatgccccatattaaaagaactcattcataggaaggtgtttcattttggtgtgcaaccctgtcattacgtcaacgcaacgtctaactggacttcccaagataaatggtaccagcgtcctcttaaaagatgccttaatccattccttgaggacagaccttagttgaaatgatagcagaatgtgcttctctctggcagctggccttctgcttctgagttgcacattaatcagattagcctgtattctcttcagtgaattttgataatggcttccagactctttggcgttggagacgcctgttaggatcttcaagtcccatcatagaaaattgaaacacagagttgttctgctgatagttttggggatacgtccatctttttaagggattgctttcatctaattctggcaggacctcaccaaaagatccagcctcatacctacatcagacaaaatatcgccgttgttccttctgtactaaagtattgtgttttgctttggaaacacccactcactttgcaatagccgtgcaagatgaatgcagattacactgatcttatgtgttacaaaattggagaaagtatttaataaaacctgttaatttttatactgacaataaaaatgtttctacagatattaatgttaacaagacaaaataaatgtcacgcaacttatttttttaataaaaaaaaaaaaaaa

SEQ ID NO: 131 - DNA, 4657 bp, Homo sapiens
  source 1..4657: mol_type = other DNA
ggcggcggctggaggagagcgcggtggagagccgagcgggcgggcggcgggtgcggagcgggcgagggagcgcgcgcggccgccacaaagctcgggcgccgcggggctgcatgcggcgtacctggcccggcgcggcgactgctctccgggctggcgggggccggccgcgagccccgggggccccgaggccgcagcttgcctgcgcgctctgagccttcgcaactcgcgagcaaagtttggtggaggcaacgccaagcctgagtcctttcttcctctcgttccccaaatccgagggcagcccgcgggcgtcatgcccgcgctcctccgcagcctggggtacgcgtgaagcccgggaggcttggcgccggcgaagacccaaggaccactcttctgcgtttggagttgctccccgcaaccccgggctcgtcgctttctccatcccgacccacgcggggcgcggggacaacacaggtcgcggaggagcgttgccattcaagtgactgcagcagcagcggcagcgcctcggttcctgagcccaccgcaggctgaaggcattgcgcgtagtccatgcccgtagaggaagtgtgcagatgggattaacgtccacatggagatatggaagaggaccggggattggtaccgtaaccatggtcagctggggtcgtttcatctgcctggtcgtggtcaccatggcaaccttgtccctggcccggccctccttcagtttagttgaggataccacattagagccagaagagccaccaaccaaataccaaatctctcaaccagaagtgtacgtggctgcgccaggggagtcgctagaggtgcgctgcctgttgaaagatgccgccgtgatcagttggactaaggatggggtgcacttggggcccaacaataggacagtgcttattggggagtacttgcagataaagggcgccacgcctagagactccggcctctatgcttgtactgccagtaggactgtagacagtgaaacttggtacttcatggtgaatgtcacagatgccatctcatccggagatgatgaggatgacaccgatggtgcggaagattttgtcagtgagaacagtaacaacaagagagcaccatactggaccaacacagaaaagatggaaaagcggctccatgctgtgcctgcggccaacactgtcaagtttcgctgcccagccggggggaacccaatgccaaccatgcggtggctgaaaaacgggaaggagtttaagcaggagcatcgcattggaggctacaaggtacgaaaccagcactggagcctcattatggaaagtgtggtcccatctgacaagggaaattatacctgtgtagtggagaatgaatacgggtccatcaatcacacgtaccacctggatgttgtggagcgatcgcctcaccggcccatcctccaagccggactgccggcaaatgcctccacagtggtcggaggagacgtagagtttgtctgcaaggtttacagtgatgcccagccccacatccagtggatcaagcacgtggaaaagaacggcagtaaatacgggcccgacgggctgccctacctcaaggttctcaagcactcggggataaatagttccaatgcagaagtgctggctctgttcaatgtgaccgaggcggatgctggggaatatatatgtaaggtctccaattatatagggcaggccaaccagtctgcctggctcactgtcctgccaaaacagcaagcgcctggaagagaaaaggagattacagcttccccagactacctggagatagccatttactgcataggggtcttcttaatcgcctgtatggtggtaacagtcatcctgtgccgaatgaagaacacgaccaagaagccagacttcagcagccagccggctgtgcacaagctgaccaaacgtatccccctgcggagacaggtaacagtttcggctgagtccagctcctccatgaactccaacaccccgctggtgaggataacaacacgcctctcttcaacggcagacacccccatgctggcaggggtctccgagtatgaacttccagaggacccaaaatgggagtttccaagagataagctgacactgggcaagcccctgggagaaggttgctttgggcaagtggtcatggcggaagcagtgggaattgacaaagacaagcccaaggaggcggtcaccgtggccgtgaagatgttgaaagatgatgccacagagaaagacctttctgatctggtgtcagagatggagatgatgaagatgattgggaaacacaagaatatcataaatcttcttggagcctgcacacaggatgggcctctctatgtcatagttgagtatgcctctaaaggcaacctccgagaatacctccgagcccggaggccacccgggatggagtactcctatgacattaaccgtgttcctgaggagcagatgaccttcaaggacttggtgtcatgcacctaccagctggccagaggcatggagtacttggcttcccaaaaatgtattcatcgagatttagcagccagaaatgttttggtaacagaaaacaatgtgatgaaaatagcagactttggactcgccagagatatcaacaatatagactattacaaaaagaccaccaatgggcggcttccagtcaagtggatggctccagaagccctgtttgatagagtatacactcatcagagtgatgtctggtccttcggggtgttaatgtgggagatcttcactttagggggctcgccctacccagggattcccgtggaggaactttttaagctgctgaaggaaggacacagaatggataagccagccaactgcaccaacgaactgtacatgatgatgagggactgttggcatgcagtgccctcccagagaccaacgttcaagcagttggtagaagacttggatcgaattctcactctcacaaccaatgaggaatacttggacctcagccaacctctcgaacagtattcacctagttaccctgacacaagaagttcttgttcttcaggagatgattctgttttttctccagaccccatgccttacgaaccatgccttcctcagtatccacacataaacggcagtgttaaaacatgaatgactgtgtctgcctgtccccaaacaggacagcactgggaacctagctacactgagcagggagaccatgcctcccagagcttgttgtctccacttgtatatatggatcagaggagtaaataattggaaaagtaatcagcatatgtgtaaagatttatacagttgaaaacttgtaatcttccccaggaggagaagaaggtttctggagcagtggactgccacaagccaccatgtaacccctctcacctgccgtgcgtactggctgtggaccagtaggactcaaggtggacgtgcgttctgccttccttgttaattttgtaataattggagaagatttatgtcagcacacacttacagagcacaaatgcagtatataggtgctggatgtatgtaaatatattcaaattatgtataaatatatattatatatttacaaggagttattttttgtattgattttaaatggatgtcccaatgcacctagaaaattggtctctctttttttaatagctatttgctaaatgctgttcttacacataatttcttaattttcaccgagcagaggtggaaaaatacttttgctttcagggaaaatggtataacgttaatttattaataaattggtaatatacaaaacaattaatcatttatagttttttttgtaatttaagtggcatttctatgcaggcagcacagcagactagttaatctattgcttggacttaactagttatcagatcctttgaaaagagaatatttacaatatatgactaatttggggaaaatgaagttttgatttatttgtgtttaaatgctgctgtcagacgattgttcttagacctcctaaatgccccatattaaaagaactcattcataggaaggtgtttcattttggtgtgcaaccctgtcattacgtcaacgcaacgtctaactggacttcccaagataaatggtaccagcgtcctcttaaaagatgccttaatccattccttgaggacagaccttagttgaaatgatagcagaatgtgcttctctctggcagctggccttctgcttctgagttgcacattaatcagattagcctgtattctcttcagtgaattttgataatggcttccagactctttggcgttggagacgcctgttaggatcttcaagtcccatcatagaaaattgaaacacagagttgttctgctgatagttttggggatacgtccatctttttaagggattgctttcatctaattctggcaggacctcaccaaaagatccagcctcatacctacatcagacaaaatatcgccgttgttccttctgtactaaagtattgtgttttgctttggaaacacccactcactttgcaatagccgtgcaagatgaatgcagattacactgatcttatgtgttacaaaattggagaaagtatttaataaaacctgttaatttttatactgacaataaaaatgtttctacagatattaatgttaacaagacaaaataaatgtcacgcaacttatttttttaataaaaaaaaaaaaaaa

SEQ ID NO: 132 - DNA, 2781 bp, Homo sapiens
  source 1..2781: mol_type = other DNA
tgactgcagcagcagcggcagcgcctcggttcctgagcccaccgcaggctgaaggcattgcgcgtagtccatgcccgtagaggaagtgtgcagatgggattaacgtccacatggagatatggaagaggaccggggattggtaccgtaaccatggtcagctggggtcgtttcatctgcctggtcgtggtcaccatggcaaccttgtccctggcccggccctccttcagtttagttgaggataccacattagagccagaagagccaccaaccaaataccaaatctctcaaccagaagtgtacgtggctgcgccaggggagtcgctagaggtgcgctgcctgttgaaagatgccgccgtgatcagttggactaaggatggggtgcacttggggcccaacaataggacagtgcttattggggagtacttgcagataaagggcgccacgcctagagactccggcctctatgcttgtactgccagtaggactgtagacagtgaaacttggtacttcatggtgaatgtcacagatgccatctcatccggagatgatgaggatgacaccgatggtgcggaagattttgtcagtgagaacagtaacaacaagagagcaccatactggaccaacacagaaaagatggaaaagcggctccatgctgtgcctgcggccaacactgtcaagtttcgctgcccagccggggggaacccaatgccaaccatgcggtggctgaaaaacgggaaggagtttaagcaggagcatcgcattggaggctacaaggtacgaaaccagcactggagcctcattatggaaagtgtggtcccatctgacaagggaaattatacctgtgtagtggagaatgaatacgggtccatcaatcacacgtaccacctggatgttgtggagcgatcgcctcaccggcccatcctccaagccggactgccggcaaatgcctccacagtggtcggaggagacgtagagtttgtctgcaaggtttacagtgatgcccagccccacatccagtggatcaagcacgtggaaaagaacggcagtaaatacgggcccgacgggctgccctacctcaaggttctcaagcactcggggataaatagttccaatgcagaagtgctggctctgttcaatgtgaccgaggcggatgctggggaatatatatgtaaggtctccaattatatagggcaggccaaccagtctgcctggctcactgtcctgccaaaacagcaagcgcctggaagagaaaaggagattacagcttccccagactacctggagatagccatttactgcataggggtcttcttaatcgcctgtatggtggtaacagtcatcctgtgccgaatgaagaacacgaccaagaagccagacttcagcagccagccggctgtgcacaagctgaccaaacgtatccccctgcggagacaggtaacagtttcggctgagtccagctcctccatgaactccaacaccccgctggtgaggataacaacacgcctctcttcaacggcagacacccccatgctggcaggggtctccgagtatgaacttccagaggacccaaaatgggagtttccaagagataagctgacactgggcaagcccctgggagaaggttgctttgggcaagtggtcatggcggaagcagtgggaattgacaaagacaagcccaaggaggcggtcaccgtggccgtgaagatgttgaaagatgatgccacagagaaagacctttctgatctggtgtcagagatggagatgatgaagatgattgggaaacacaagaatatcataaatcttcttggagcctgcacacaggatgggcctctctatgtcatagttgagtatgcctctaaaggcaacctccgagaatacctccgagcccggaggccacccgggatggagtactcctatgacattaaccgtgttcctgaggagcagatgaccttcaaggacttggtgtcatgcacctaccagctggccagaggcatggagtacttggcttcccaaaaatgtattcatcgagatttagcagccagaaatgttttggtaacagaaaacaatgtgatgaaaatagcagactttggactcgccagagatatcaacaatatagactattacaaaaagaccaccaatgggcggcttccagtcaagtggatggctccagaagccctgtttgatagagtatacactcatcagagtgatgtctggtccttcggggtgttaatgtgggagatcttcactttagggggctcgccctacccagggattcccgtggaggaactttttaagctgctgaaggaaggacacagaatggataagccagccaactgcaccaacgaactgtacatgatgatgagggactgttggcatgcagtgccctcccagagaccaacgttcaagcagttggtagaagacttggatcgaattctcactctcacaaccaatgagatctgaaagtttatggcttcattgagaaactgggaaaagttggtcaggcgcagtggctcatgcctgtaatcccagcactttgggaggccgaggcaggcggatcatgaggtcaggagttccagaccagcctggccaacatggtgaaaccctgtctctactaaagatacaaaaaattagccgggcgtgttggtgtgcacctgtaatcccagctactccgggaggctgaggcaggagagtcacttgaaccggggaggcggaggttgcagtgagccgagatcatgccattgcattccagccttggcgacagagcgagactccgtctcaaaa

SEQ ID NO: 133 - DNA, 3821 bp, Homo sapiens
  source 1..3821: mol_type = other DNA
tgactgcagcagcagcggcagcgcctcggttcctgagcccaccgcaggctgaaggcattgcgcgtagtccatgcccgtagaggaagtgtgcagatgggattaacgtccacatggagatatggaagaggaccggggattggtaccgtaaccatggtcagctggggtcgtttcatctgcctggtcgtggtcaccatggcaaccttgtccctggcccggccctccttcagtttagttgaggataccacattagagccagaagagccaccaaccaaataccaaatctctcaaccagaagtgtacgtggctgcgccaggggagtcgctagaggtgcgctgcctgttgaaagatgccgccgtgatcagttggactaaggatggggtgcacttggggcccaacaataggacagtgcttattggggagtacttgcagataaagggcgccacgcctagagactccggcctctatgcttgtactgccagtaggactgtagacagtgaaacttggtacttcatggtgaatgtcacagatgccatctcatccggagatgatgaggatgacaccgatggtgcggaagattttgtcagtgagaacagtaacaacaagagagcaccatactggaccaacacagaaaagatggaaaagcggctccatgctgtgcctgcggccaacactgtcaagtttcgctgcccagccggggggaacccaatgccaaccatgcggtggctgaaaaacgggaaggagtttaagcaggagcatcgcattggaggctacaaggtacgaaaccagcactggagcctcattatggaaagtgtggtcccatctgacaagggaaattatacctgtgtagtggagaatgaatacgggtccatcaatcacacgtaccacctggatgttgtggcgcctggaagagaaaaggagattacagcttccccagactacctggagatagccatttactgcataggggtcttcttaatcgcctgtatggtggtaacagtcatcctgtgccgaatgaagaacacgaccaagaagccagacttcagcagccagccggctgtgcacaagctgaccaaacgtatccccctgcggagacaggtaacagtttcggctgagtccagctcctccatgaactccaacaccccgctggtgaggataacaacacgcctctcttcaacggcagacacccccatgctggcaggggtctccgagtatgaacttccagaggacccaaaatgggagtttccaagagataagctgacactgggcaagcccctgggagaaggttgctttgggcaagtggtcatggcggaagcagtgggaattgacaaagacaagcccaaggaggcggtcaccgtggccgtgaagatgttgaaagatgatgccacagagaaagacctttctgatctggtgtcagagatggagatgatgaagatgattgggaaacacaagaatatcataaatcttcttggagcctgcacacaggatgggcctctctatgtcatagttgagtatgcctctaaaggcaacctccgagaatacctccgagcccggaggccacccgggatggagtactcctatgacattaaccgtgttcctgaggagcagatgaccttcaaggacttggtgtcatgcacctaccagctggccagaggcatggagtacttggcttcccaaaaatgtattcatcgagatttagcagccagaaatgttttggtaacagaaaacaatgtgatgaaaatagcagactttggactcgccagagatatcaacaatatagactattacaaaaagaccaccaatgggcggcttccagtcaagtggatggctccagaagccctgtttgatagagtatacactcatcagagtgatgtctggtccttcggggtgttaatgtgggagatcttcactttagggggctcgccctacccagggattcccgtggaggaactttttaagctgctgaaggaaggacacagaatggataagccagccaactgcaccaacgaactgtacatgatgatgagggactgttggcatgcagtgccctcccagagaccaacgttcaagcagttggtagaagacttggatcgaattctcactctcacaaccaatgaggaatacttggacctcagccaacctctcgaacagtattcacctagttaccctgacacaagaagttcttgttcttcaggagatgattctgttttttctccagaccccatgccttacgaaccatgccttcctcagtatccacacataaacggcagtgttaaaacatgaatgactgtgtctgcctgtccccaaacaggacagcactgggaacctagctacactgagcagggagaccatgcctcccagagcttgttgtctccacttgtatatatggatcagaggagtaaataattggaaaagtaatcagcatatgtgtaaagatttatacagttgaaaacttgtaatcttccccaggaggagaagaaggtttctggagcagtggactgccacaagccaccatgtaacccctctcacctgccgtgcgtactggctgtggaccagtaggactcaaggtggacgtgcgttctgccttccttgttaattttgtaataattggagaagatttatgtcagcacacacttacagagcacaaatgcagtatataggtgctggatgtatgtaaatatattcaaattatgtataaatatatattatatatttacaaggagttattttttgtattgattttaaatggatgtcccaatgcacctagaaaattggtctctctttttttaatagctatttgctaaatgctgttcttacacataatttcttaattttcaccgagcagaggtggaaaaatacttttgctttcagggaaaatggtataacgttaatttattaataaattggtaatatacaaaacaattaatcatttatagttttttttgtaatttaagtggcatttctatgcaggcagcacagcagactagttaatctattgcttggacttaactagttatcagatcctttgaaaagagaatatttacaatatatgactaatttggggaaaatgaagttttgatttatttgtgtttaaatgctgctgtcagacgattgttcttagacctcctaaatgccccatattaaaagaactcattcataggaaggtgtttcattttggtgtgcaaccctgtcattacgtcaacgcaacgtctaactggacttcccaagataaatggtaccagcgtcctcttaaaagatgccttaatccattccttgaggacagaccttagttgaaatgatagcagaatgtgcttctctctggcagctggccttctgcttctgagttgcacattaatcagattagcctgtattctcttcagtgaattttgataatggcttccagactctttggcgttggagacgcctgttaggatcttcaagtcccatcatagaaaattgaaacacagagttgttctgctgatagttttggggatacgtccatctttttaagggattgctttcatctaattctggcaggacctcaccaaaagatccagcctcatacctacatcagacaaaatatcgccgttgttccttctgtactaaagtattgtgttttgctttggaaacacccactcactttgcaatagccgtgcaagatgaatgcagattacactgatcttatgtgttacaaaattggagaaagtatttaataaaacctgttaatttttatactgacaataaaaatgtttctacagatattaatgttaacaagacaaaataaatgtcacgcaacttatttttttaataaaaaaaaaaaaaaa

SEQ ID NO: 134 - DNA, 3708 bp, Homo sapiens
  source 1..3708: mol_type = other DNA
aatttgttgaggaatttccccctagccttgaccccttgacagctcccgctcctactcagtgctggggagaagtagggaggccttaagcgaagagatgggtctgcactttggaggagccggacactgttgactttcctgatgtgaaatctacccaggaacaaaacaccagtgactgcagcagcagcggcagcgcctcggttcctgagcccaccgcaggctgaaggcattgcgcgtagtccatgcccgtagaggaagtgtgcagatgggattaacgtccacatggagatatggaagaggaccggggattggtaccgtaaccatggtcagctggggtcgtttcatctgcctggtcgtggtcaccatggcaaccttgtccctggcccggccctccttcagtttagttgaggataccacattagagccagaagatgccatctcatccggagatgatgaggatgacaccgatggtgcggaagattttgtcagtgagaacagtaacaacaagagagcaccatactggaccaacacagaaaagatggaaaagcggctccatgctgtgcctgcggccaacactgtcaagtttcgctgcccagccggggggaacccaatgccaaccatgcggtggctgaaaaacgggaaggagtttaagcaggagcatcgcattggaggctacaaggtacgaaaccagcactggagcctcattatggaaagtgtggtcccatctgacaagggaaattatacctgtgtagtggagaatgaatacgggtccatcaatcacacgtaccacctggatgttgtggagcgatcgcctcaccggcccatcctccaagccggactgccggcaaatgcctccacagtggtcggaggagacgtagagtttgtctgcaaggtttacagtgatgcccagccccacatccagtggatcaagcacgtggaaaagaacggcagtaaatacgggcccgacgggctgccctacctcaaggttctcaaggccgccggtgttaacaccacggacaaagagattgaggttctctatattcggaatgtaacttttgaggacgctggggaatatacgtgcttggcgggtaattctattgggatatcctttcactctgcatggttgacagttctgccagcgcctggaagagaaaaggagattacagcttccccagactacctggagatagccatttactgcataggggtcttcttaatcgcctgtatggtggtaacagtcatcctgtgccgaatgaagaacacgaccaagaagccagacttcagcagccagccggctgtgcacaagctgaccaaacgtatccccctgcggagacaggtaacagtttcggctgagtccagctcctccatgaactccaacaccccgctggtgaggataacaacacgcctctcttcaacggcagacacccccatgctggcaggggtctccgagtatgaacttccagaggacccaaaatgggagtttccaagagataagctgacactgggcaagcccctgggagaaggttgctttgggcaagtggtcatggcggaagcagtgggaattgacaaagacaagcccaaggaggcggtcaccgtggccgtgaagatgttgaaagatgatgccacagagaaagacctttctgatctggtgtcagagatggagatgatgaagatgattgggaaacacaagaatatcataaatcttcttggagcctgcacacaggatgggcctctctatgtcatagttgagtatgcctctaaaggcaacctccgagaatacctccgagcccggaggccacccgggatggagtactcctatgacattaaccgtgttcctgaggagcagatgaccttcaaggacttggtgtcatgcacctaccagctggccagaggcatggagtacttggcttcccaaaaatgtattcatcgagatttagcagccagaaatgttttggtaacagaaaacaatgtgatgaaaatagcagactttggactcgccagagatatcaacaatatagactattacaaaaagaccaccaatgggcggcttccagtcaagtggatggctccagaagccctgtttgatagagtatacactcatcagagtgatgtctggtccttcggggtgttaatgtgggagatcttcactttagggggctcgccctacccagggattcccgtggaggaactttttaagctgctgaaggaaggacacagaatggataagccagccaactgcaccaacgaactgtacatgatgatgagggactgttggcatgcagtgccctcccagagaccaacgttcaagcagttggtagaagacttggatcgaattctcactctcacaaccaatgaggaggagaagaaggtttctggagcagtggactgccacaagccaccatgtaacccctctcacctgccgtgcgtactggctgtggaccagtaggactcaaggtggacgtgcgttctgccttccttgttaattttgtaataattggagaagatttatgtcagcacacacttacagagcacaaatgcagtatataggtgctggatgtatgtaaatatattcaaattatgtataaatatatattatatatttacaaggagttattttttgtattgattttaaatggatgtcccaatgcacctagaaaattggtctctctttttttaatagctatttgctaaatgctgttcttacacataatttcttaattttcaccgagcagaggtggaaaaatacttttgctttcagggaaaatggtataacgttaatttattaataaattggtaatatacaaaacaattaatcatttatagttttttttgtaatttaagtggcatttctatgcaggcagcacagcagactagttaatctattgcttggacttaactagttatcagatcctttgaaaagagaatatttacaatatatgactaatttggggaaaatgaagttttgatttatttgtgtttaaatgctgctgtcagacgattgttcttagacctcctaaatgccccatattaaaagaactcattcataggaaggtgtttcattttggtgtgcaaccctgtcattacgtcaacgcaacgtctaactggacttcccaagataaatggtaccagcgtcctcttaaaagatgccttaatccattccttgaggacagaccttagttgaaatgatagcagaatgtgcttctctctggcagctggccttctgcttctgagttgcacattaatcagattagcctgtattctcttcagtgaattttgataatggcttccagactctttggcgttggagacgcctgttaggatcttcaagtcccatcatagaaaattgaaacacagagttgttctgctgatagttttggggatacgtccatctttttaagggattgctttcatctaattctggcaggacctcaccaaaagatccagcctcatacctacatcagacaaaatatcgccgttgttccttctgtactaaagtattgtgttttgctttggaaacacccactcactttgcaatagccgtgcaagatgaatgcagattacactgatcttatgtgttacaaaattggagaaagtatttaataaaacctgttaatttttatactgacaataaaaatgtttctacagatattaatgttaacaagacaaaataaatgtcacgcaacttatttttttaataaaaaaaaaaaaaaa

SEQ ID NO: 135 - DNA, 4103 bp, Homo sapiens
  source 1..4103: mol_type = other DNA
gagcacacattgcctcactgaagtggctgcacgtatctgagtcctgtagctactgttttatctctgtttcttaaaagtatgcttttaaaaagattagcctcacacatttctgtggaccggtctggtggtatcacctgggactctgaggtgaggatggaaggatttagcagataatgaaaaagaactctgtttgcgcacatttgagaggctgaaaaatggttttatcccacttgggctggagtgatttggcattggggaagattccctgactcgccaatctctttcctttagtgactgcagcagcagcggcagcgcctcggttcctgagcccaccgcaggctgaaggcattgcgcgtagtccatgcccgtagaggaagtgtgcagatgggattaacgtccacatggagatatggaagaggaccggggattggtaccgtaaccatggtcagctggggtcgtttcatctgcctggtcgtggtcaccatggcaaccttgtccctggcccggccctccttcagtttagttgaggataccacattagagccagaaggagcaccatactggaccaacacagaaaagatggaaaagcggctccatgctgtgcctgcggccaacactgtcaagtttcgctgcccagccggggggaacccaatgccaaccatgcggtggctgaaaaacgggaaggagtttaagcaggagcatcgcattggaggctacaaggtacgaaaccagcactggagcctcattatggaaagtgtggtcccatctgacaagggaaattatacctgtgtagtggagaatgaatacgggtccatcaatcacacgtaccacctggatgttgtggagcgatcgcctcaccggcccatcctccaagccggactgccggcaaatgcctccacagtggtcggaggagacgtagagtttgtctgcaaggtttacagtgatgcccagccccacatccagtggatcaagcacgtggaaaagaacggcagtaaatacgggcccgacgggctgccctacctcaaggttctcaaggccgccggtgttaacaccacggacaaagagattgaggttctctatattcggaatgtaacttttgaggacgctggggaatatacgtgcttggcgggtaattctattgggatatcctttcactctgcatggttgacagttctgccagcgcctggaagagaaaaggagattacagcttccccagactacctggagatagccatttactgcataggggtcttcttaatcgcctgtatggtggtaacagtcatcctgtgccgaatgaagaacacgaccaagaagccagacttcagcagccagccggctgtgcacaagctgaccaaacgtatccccctgcggagacaggtaacagtttcggctgagtccagctcctccatgaactccaacaccccgctggtgaggataacaacacgcctctcttcaacggcagacacccccatgctggcaggggtctccgagtatgaacttccagaggacccaaaatgggagtttccaagagataagctgacactgggcaagcccctgggagaaggttgctttgggcaagtggtcatggcggaagcagtgggaattgacaaagacaagcccaaggaggcggtcaccgtggccgtgaagatgttgaaagatgatgccacagagaaagacctttctgatctggtgtcagagatggagatgatgaagatgattgggaaacacaagaatatcataaatcttcttggagcctgcacacaggatgggcctctctatgtcatagttgagtatgcctctaaaggcaacctccgagaatacctccgagcccggaggccacccgggatggagtactcctatgacattaaccgtgttcctgaggagcagatgaccttcaaggacttggtgtcatgcacctaccagctggccagaggcatggagtacttggcttcccaaaaatgtattcatcgagatttagcagccagaaatgttttggtaacagaaaacaatgtgatgaaaatagcagactttggactcgccagagatatcaacaatatagactattacaaaaagaccaccaatgggcggcttccagtcaagtggatggctccagaagccctgtttgatagagtatacactcatcagagtgatgtctggtccttcggggtgttaatgtgggagatcttcactttagggggctcgccctacccagggattcccgtggaggaactttttaagctgctgaaggaaggacacagaatggataagccagccaactgcaccaacgaactgtacatgatgatgagggactgttggcatgcagtgccctcccagagaccaacgttcaagcagttggtagaagacttggatcgaattctcactctcacaaccaatgaggaatacttggacctcagccaacctctcgaacagtattcacctagttaccctgacacaagaagttcttgttcttcaggagatgattctgttttttctccagaccccatgccttacgaaccatgccttcctcagtatccacacataaacggcagtgttaaaacatgaatgactgtgtctgcctgtccccaaacaggacagcactgggaacctagctacactgagcagggagaccatgcctcccagagcttgttgtctccacttgtatatatggatcagaggagtaaataattggaaaagtaatcagcatatgtgtaaagatttatacagttgaaaacttgtaatcttccccaggaggagaagaaggtttctggagcagtggactgccacaagccaccatgtaacccctctcacctgccgtgcgtactggctgtggaccagtaggactcaaggtggacgtgcgttctgccttccttgttaattttgtaataattggagaagatttatgtcagcacacacttacagagcacaaatgcagtatataggtgctggatgtatgtaaatatattcaaattatgtataaatatatattatatatttacaaggagttattttttgtattgattttaaatggatgtcccaatgcacctagaaaattggtctctctttttttaatagctatttgctaaatgctgttcttacacataatttcttaattttcaccgagcagaggtggaaaaatacttttgctttcagggaaaatggtataacgttaatttattaataaattggtaatatacaaaacaattaatcatttatagttttttttgtaatttaagtggcatttctatgcaggcagcacagcagactagttaatctattgcttggacttaactagttatcagatcctttgaaaagagaatatttacaatatatgactaatttggggaaaatgaagttttgatttatttgtgtttaaatgctgctgtcagacgattgttcttagacctcctaaatgccccatattaaaagaactcattcataggaaggtgtttcattttggtgtgcaaccctgtcattacgtcaacgcaacgtctaactggacttcccaagataaatggtaccagcgtcctcttaaaagatgccttaatccattccttgaggacagaccttagttgaaatgatagcagaatgtgcttctctctggcagctggccttctgcttctgagttgcacattaatcagattagcctgtattctcttcagtgaattttgataatggcttccagactctttggcgttggagacgcctgttaggatcttcaagtcccatcatagaaaattgaaacacagagttgttctgctgatagttttggggatacgtccatctttttaagggattgctttcatctaattctggcaggacctcaccaaaagatccagcctcatacctacatcagacaaaatatcgccgttgttccttctgtactaaagtattgtgttttgctttggaaacacccactcactttgcaatagccgtgcaagatgaatgcagattacactgatcttatgtgttacaaaattggagaaagtatttaataaaacctgttaatttttatactgacaataaaaatgtttctacagatattaatgttaacaagacaaaataaatgtcacgcaacttatttttttaataaaaaaaaaaaaaaa

SEQ ID NO: 136 - DNA, 4306 bp, Homo sapiens
  source 1..4306: mol_type = other DNA
ggcggcggctggaggagagcgcggtggagagccgagcgggcgggcggcgggtgcggagcgggcgagggagcgcgcgcggccgccacaaagctcgggcgccgcggggctgcatgcggcgtacctggcccggcgcggcgactgctctccgggctggcgggggccggccgcgagccccgggggccccgaggccgcagcttgcctgcgcgctctgagccttcgcaactcgcgagcaaagtttggtggaggcaacgccaagcctgagtcctttcttcctctcgttccccaaatccgagggcagcccgcgggcgtcatgcccgcgctcctccgcagcctggggtacgcgtgaagcccgggaggcttggcgccggcgaagacccaaggaccactcttctgcgtttggagttgctccccgcaaccccgggctcgtcgctttctccatcccgacccacgcggggcgcggggacaacacaggtcgcggaggagcgttgccattcaagtgactgcagcagcagcggcagcgcctcggttcctgagcccaccgcaggctgaaggcattgcgcgtagtccatgcccgtagaggaagtgtgcagatgggattaacgtccacatggagatatggaagaggaccggggattggtaccgtaaccatggtcagctggggtcgtttcatctgcctggtcgtggtcaccatggcaaccttgtccctggcccggccctccttcagtttagttgaggataccacattagagccagaagagccaccaaccaaataccaaatctctcaaccagaagtgtacgtggctgcgccaggggagtcgctagaggtgcgctgcctgttgaaagatgccgccgtgatcagttggactaaggatggggtgcacttggggcccaacaataggacagtgcttattggggagtacttgcagataaagggcgccacgcctagagactccggcctctatgcttgtactgccagtaggactgtagacagtgaaacttggtacttcatggtgaatgtcacagatgccatctcatccggagatgatgaggatgacaccgatggtgcggaagattttgtcagtgagaacagtaacaacaagagagcaccatactggaccaacacagaaaagatggaaaagcggctccatgctgtgcctgcggccaacactgtcaagtttcgctgcccagccggggggaacccaatgccaaccatgcggtggctgaaaaacgggaaggagtttaagcaggagcatcgcattggaggctacaaggtacgaaaccagcactggagcctcattatggaaagtgtggtcccatctgacaagggaaattatacctgtgtagtggagaatgaatacgggtccatcaatcacacgtaccacctggatgttgtggagcgatcgcctcaccggcccatcctccaagccggactgccggcaaatgcctccacagtggtcggaggagacgtagagtttgtctgcaaggtttacagtgatgcccagccccacatccagtggatcaagcacgtggaaaagaacggcagtaaatacgggcccgacgggctgccctacctcaaggttctcaaggtttcggctgagtccagctcctccatgaactccaacaccccgctggtgaggataacaacacgcctctcttcaacggcagacacccccatgctggcaggggtctccgagtatgaacttccagaggacccaaaatgggagtttccaagagataagctgacactgggcaagcccctgggagaaggttgctttgggcaagtggtcatggcggaagcagtgggaattgacaaagacaagcccaaggaggcggtcaccgtggccgtgaagatgttgaaagatgatgccacagagaaagacctttctgatctggtgtcagagatggagatgatgaagatgattgggaaacacaagaatatcataaatcttcttggagcctgcacacaggatgggcctctctatgtcatagttgagtatgcctctaaaggcaacctccgagaatacctccgagcccggaggccacccgggatggagtactcctatgacattaaccgtgttcctgaggagcagatgaccttcaaggacttggtgtcatgcacctaccagctggccagaggcatggagtacttggcttcccaaaaatgtattcatcgagatttagcagccagaaatgttttggtaacagaaaacaatgtgatgaaaatagcagactttggactcgccagagatatcaacaatatagactattacaaaaagaccaccaatgggcggcttccagtcaagtggatggctccagaagccctgtttgatagagtatacactcatcagagtgatgtctggtccttcggggtgttaatgtgggagatcttcactttagggggctcgccctacccagggattcccgtggaggaactttttaagctgctgaaggaaggacacagaatggataagccagccaactgcaccaacgaactgtacatgatgatgagggactgttggcatgcagtgccctcccagagaccaacgttcaagcagttggtagaagacttggatcgaattctcactctcacaaccaatgaggaatacttggacctcagccaacctctcgaacagtattcacctagttaccctgacacaagaagttcttgttcttcaggagatgattctgttttttctccagaccccatgccttacgaaccatgccttcctcagtatccacacataaacggcagtgttaaaacatgaatgactgtgtctgcctgtccccaaacaggacagcactgggaacctagctacactgagcagggagaccatgcctcccagagcttgttgtctccacttgtatatatggatcagaggagtaaataattggaaaagtaatcagcatatgtgtaaagatttatacagttgaaaacttgtaatcttccccaggaggagaagaaggtttctggagcagtggactgccacaagccaccatgtaacccctctcacctgccgtgcgtactggctgtggaccagtaggactcaaggtggacgtgcgttctgccttccttgttaattttgtaataattggagaagatttatgtcagcacacacttacagagcacaaatgcagtatataggtgctggatgtatgtaaatatattcaaattatgtataaatatatattatatatttacaaggagttattttttgtattgattttaaatggatgtcccaatgcacctagaaaattggtctctctttttttaatagctatttgctaaatgctgttcttacacataatttcttaattttcaccgagcagaggtggaaaaatacttttgctttcagggaaaatggtataacgttaatttattaataaattggtaatatacaaaacaattaatcatttatagttttttttgtaatttaagtggcatttctatgcaggcagcacagcagactagttaatctattgcttggacttaactagttatcagatcctttgaaaagagaatatttacaatatatgactaatttggggaaaatgaagttttgatttatttgtgtttaaatgctgctgtcagacgattgttcttagacctcctaaatgccccatattaaaagaactcattcataggaaggtgtttcattttggtgtgcaaccctgtcattacgtcaacgcaacgtctaactggacttcccaagataaatggtaccagcgtcctcttaaaagatgccttaatccattccttgaggacagaccttagttgaaatgatagcagaatgtgcttctctctggcagctggccttctgcttctgagttgcacattaatcagattagcctgtattctcttcagtgaattttgataatggcttccagactctttggcgttggagacgcctgttaggatcttcaagtcccatcatagaaaattgaaacacagagttgttctgctgatagttttggggatacgtccatctttttaagggattgctttcatctaattctggcaggacctcaccaaaagatccagcctcatacctacatcagacaaaatatcgccgttgttccttctgtactaaagtattgtgttttgctttggaaacacccactcactttgcaatagccgtgcaagatgaatgcagattacactgatcttatgtgttacaaaattggagaaagtatttaataaaacctgttaatttttatactgacaataaaaatgtttctacagatattaatgttaacaagacaaaataaatgtcacgcaacttatttttttaataaaaaaaaaaaaaaa

SEQ ID NO: 137 - DNA, 4303 bp, Homo sapiens
  source 1..4303: mol_type = other DNA
ggcggcggctggaggagagcgcggtggagagccgagcgggcgggcggcgggtgcggagcgggcgagggagcgcgcgcggccgccacaaagctcgggcgccgcggggctgcatgcggcgtacctggcccggcgcggcgactgctctccgggctggcgggggccggccgcgagccccgggggccccgaggccgcagcttgcctgcgcgctctgagccttcgcaactcgcgagcaaagtttggtggaggcaacgccaagcctgagtcctttcttcctctcgttccccaaatccgagggcagcccgcgggcgtcatgcccgcgctcctccgcagcctggggtacgcgtgaagcccgggaggcttggcgccggcgaagacccaaggaccactcttctgcgtttggagttgctccccgcaaccccgggctcgtcgctttctccatcccgacccacgcggggcgcggggacaacacaggtcgcggaggagcgttgccattcaagtgactgcagcagcagcggcagcgcctcggttcctgagcccaccgcaggctgaaggcattgcgcgtagtccatgcccgtagaggaagtgtgcagatgggattaacgtccacatggagatatggaagaggaccggggattggtaccgtaaccatggtcagctggggtcgtttcatctgcctggtcgtggtcaccatggcaaccttgtccctggcccggccctccttcagtttagttgaggataccacattagagccagaaggagcaccatactggaccaacacagaaaagatggaaaagcggctccatgctgtgcctgcggccaacactgtcaagtttcgctgcccagccggggggaacccaatgccaaccatgcggtggctgaaaaacgggaaggagtttaagcaggagcatcgcattggaggctacaaggtacgaaaccagcactggagcctcattatggaaagtgtggtcccatctgacaagggaaattatacctgtgtagtggagaatgaatacgggtccatcaatcacacgtaccacctggatgttgtggagcgatcgcctcaccggcccatcctccaagccggactgccggcaaatgcctccacagtggtcggaggagacgtagagtttgtctgcaaggtttacagtgatgcccagccccacatccagtggatcaagcacgtggaaaagaacggcagtaaatacgggcccgacgggctgccctacctcaaggttctcaaggccgccggtgttaacaccacggacaaagagattgaggttctctatattcggaatgtaacttttgaggacgctggggaatatacgtgcttggcgggtaattctattgggatatcctttcactctgcatggttgacagttctgccagcgcctggaagagaaaaggagattacagcttccccagactacctggagatagccatttactgcataggggtcttcttaatcgcctgtatggtggtaacagtcatcctgtgccgaatgaagaacacgaccaagaagccagacttcagcagccagccggctgtgcacaagctgaccaaacgtatccccctgcggagacaggtttcggctgagtccagctcctccatgaactccaacaccccgctggtgaggataacaacacgcctctcttcaacggcagacacccccatgctggcaggggtctccgagtatgaacttccagaggacccaaaatgggagtttccaagagataagctgacactgggcaagcccctgggagaaggttgctttgggcaagtggtcatggcggaagcagtgggaattgacaaagacaagcccaaggaggcggtcaccgtggccgtgaagatgttgaaagatgatgccacagagaaagacctttctgatctggtgtcagagatggagatgatgaagatgattgggaaacacaagaatatcataaatcttcttggagcctgcacacaggatgggcctctctatgtcatagttgagtatgcctctaaaggcaacctccgagaatacctccgagcccggaggccacccgggatggagtactcctatgacattaaccgtgttcctgaggagcagatgaccttcaaggacttggtgtcatgcacctaccagctggccagaggcatggagtacttggcttcccaaaaatgtattcatcgagatttagcagccagaaatgttttggtaacagaaaacaatgtgatgaaaatagcagactttggactcgccagagatatcaacaatatagactattacaaaaagaccaccaatgggcggcttccagtcaagtggatggctccagaagccctgtttgatagagtatacactcatcagagtgatgtctggtccttcggggtgttaatgtgggagatcttcactttagggggctcgccctacccagggattcccgtggaggaactttttaagctgctgaaggaaggacacagaatggataagccagccaactgcaccaacgaactgtacatgatgatgagggactgttggcatgcagtgccctcccagagaccaacgttcaagcagttggtagaagacttggatcgaattctcactctcacaaccaatgaggaatacttggacctcagccaacctctcgaacagtattcacctagttaccctgacacaagaagttcttgttcttcaggagatgattctgttttttctccagaccccatgccttacgaaccatgccttcctcagtatccacacataaacggcagtgttaaaacatgaatgactgtgtctgcctgtccccaaacaggacagcactgggaacctagctacactgagcagggagaccatgcctcccagagcttgttgtctccacttgtatatatggatcagaggagtaaataattggaaaagtaatcagcatatgtgtaaagatttatacagttgaaaacttgtaatcttccccaggaggagaagaaggtttctggagcagtggactgccacaagccaccatgtaacccctctcacctgccgtgcgtactggctgtggaccagtaggactcaaggtggacgtgcgttctgccttccttgttaattttgtaataattggagaagatttatgtcagcacacacttacagagcacaaatgcagtatataggtgctggatgtatgtaaatatattcaaattatgtataaatatatattatatatttacaaggagttattttttgtattgattttaaatggatgtcccaatgcacctagaaaattggtctctctttttttaatagctatttgctaaatgctgttcttacacataatttcttaattttcaccgagcagaggtggaaaaatacttttgctttcagggaaaatggtataacgttaatttattaataaattggtaatatacaaaacaattaatcatttatagttttttttgtaatttaagtggcatttctatgcaggcagcacagcagactagttaatctattgcttggacttaactagttatcagatcctttgaaaagagaatatttacaatatatgactaatttggggaaaatgaagttttgatttatttgtgtttaaatgctgctgtcagacgattgttcttagacctcctaaatgccccatattaaaagaactcattcataggaaggtgtttcattttggtgtgcaaccctgtcattacgtcaacgcaacgtctaactggacttcccaagataaatggtaccagcgtcctcttaaaagatgccttaatccattccttgaggacagaccttagttgaaatgatagcagaatgtgcttctctctggcagctggccttctgcttctgagttgcacattaatcagattagcctgtattctcttcagtgaattttgataatggcttccagactctttggcgttggagacgcctgttaggatcttcaagtcccatcatagaaaattgaaacacagagttgttctgctgatagttttggggatacgtccatctttttaagggattgctttcatctaattctggcaggacctcaccaaaagatccagcctcatacctacatcagacaaaatatcgccgttgttccttctgtactaaagtattgtgttttgctttggaaacacccactcactttgcaatagccgtgcaagatgaatgcagattacactgatcttatgtgttacaaaattggagaaagtatttaataaaacctgttaatttttatactgacaataaaaatgtttctacagatattaatgttaacaagacaaaataaatgtcacgcaacttatttttttaataaaaaaaaaaaaaaa

SEQ ID NO: 138 - DNA, 3011 bp, Homo sapiens
  source 1..3011: mol_type = other DNA
ggcggcggctggaggagagcgcggtggagagccgagcgggcgggcggcgggtgcggagcgggcgagggagcgcgcgcggccgccacaaagctcgggcgccgcggggctgcatgcggcgtacctggcccggcgcggcgactgctctccgggctggcgggggccggccgcgagccccgggggccccgaggccgcagcttgcctgcgcgctctgagccttcgcaactcgcgagcaaagtttggtggaggcaacgccaagcctgagtcctttcttcctctcgttccccaaatccgagggcagcccgcgggcgtcatgcccgcgctcctccgcagcctggggtacgcgtgaagcccgggaggcttggcgccggcgaagacccaaggaccactcttctgcgtttggagttgctccccgcaaccccgggctcgtcgctttctccatcccgacccacgcggggcgcggggacaacacaggtcgcggaggagcgttgccattcaagtgactgcagcagcagcggcagcgcctcggttcctgagcccaccgcaggctgaaggcattgcgcgtagtccatgcccgtagaggaagtgtgcagatgggattaacgtccacatggagatatggaagaggaccggggattggtaccgtaaccatggtcagctggggtcgtttcatctgcctggtcgtggtcaccatggcaaccttgtccctggcccggccctccttcagtttagttgaggataccacattagagccagaagatgccatctcatccggagatgatgaggatgacaccgatggtgcggaagattttgtcagtgagaacagtaacaacaagagagcaccatactggaccaacacagaaaagatggaaaagcggctccatgctgtgcctgcggccaacactgtcaagtttcgctgcccagccggggggaacccaatgccaaccatgcggtggctgaaaaacgggaaggagtttaagcaggagcatcgcattggaggctacaaggtacgaaaccagcactggagcctcattatggaaagtgtggtcccatctgacaagggaaattatacctgtgtagtggagaatgaatacgggtccatcaatcacacgtaccacctggatgttgtggagcgatcgcctcaccggcccatcctccaagccggactgccggcaaatgcctccacagtggtcggaggagacgtagagtttgtctgcaaggtttacagtgatgcccagccccacatccagtggatcaagcacgtggaaaagaacggcagtaaatacgggcccgacgggctgccctacctcaaggttctcaagcactcggggataaatagttccaatgcagaagtgctggctctgttcaatgtgaccgaggcggatgctggggaatatatatgtaaggtctccaattatatagggcaggccaaccagtctgcctggctcactgtcctgccaaaacagcaagcgcctggaagagaaaaggagattacagcttccccagactacctggagatagccatttactgcataggggtcttcttaatcgcctgtatggtggtaacagtcatcctgtgccgaatgaagaacacgaccaagaagccagacttcagcagccagccggctgtgcacaagctgaccaaacgtatccccctgcggagacaggtaacagtttcggctgagtccagctcctccatgaactccaacaccccgctggtgaggataacaacacgcctctcttcaacggcagacacccccatgctggcaggggtctccgagtatgaacttccagaggacccaaaatgggagtttccaagagataagctgacactgggcaagcccctgggagaaggttgctttgggcaagtggtcatggcggaagcagtgggaattgacaaagacaagcccaaggaggcggtcaccgtggccgtgaagatgttgaaagatgatgccacagagaaagacctttctgatctggtgtcagagatggagatgatgaagatgattgggaaacacaagaatatcataaatcttcttggagcctgcacacaggatgggcctctctatgtcatagttgagtatgcctctaaaggcaacctccgagaatacctccgagcccggaggccacccgggatggagtactcctatgacattaaccgtgttcctgaggagcagatgaccttcaaggacttggtgtcatgcacctaccagctggccagaggcatggagtacttggcttcccaaaaatgtattcatcgagatttagcagccagaaatgttttggtaacagaaaacaatgtgatgaaaatagcagactttggactcgccagagatatcaacaatatagactattacaaaaagaccaccaatgggcggcttccagtcaagtggatggctccagaagccctgtttgatagagtatacactcatcagagtgatgtctggtccttcggggtgttaatgtgggagatcttcactttagggggctcgccctacccagggattcccgtggaggaactttttaagctgctgaaggaaggacacagaatggataagccagccaactgcaccaacgaactgtacatgatgatgagggactgttggcatgcagtgccctcccagagaccaacgttcaagcagttggtagaagacttggatcgaattctcactctcacaaccaatgagatctgaaagtttatggcttcattgagaaactgggaaaagttggtcaggcgcagtggctcatgcctgtaatcccagcactttgggaggccgaggcaggcggatcatgaggtcaggagttccagaccagcctggccaacatggtgaaaccctgtctctactaaagatacaaaaaattagccgggcgtgttggtgtgcacctgtaatcccagctactccgggaggctgaggcaggagagtcacttgaaccggggaggcggaggttgcagtgagccgagatcatgccattgcattccagccttggcgacagagcgagactccgtctcaaaa

SEQ ID NO: 139 - DNA, 4286 bp, Homo sapiens
  source 1..4286: mol_type = other DNA
gtcgcgggcagctggcgccgcgcggtcctgctctgccggtcgcacggacgcaccggcgggccgccggccggagggacggggcgggagctgggcccgcggacagcgagccggagcgggagccgcgcgtagcgagccgggctccggcgctcgccagtctcccgagcggcgcccgcctcccgccggtgcccgcgccgggccgtggggggcagcatgcccgcgcgcgctgcctgaggacgccgcggcccccgcccccgccatgggcgcccctgcctgcgccctcgcgctctgcgtggccgtggccatcgtggccggcgcctcctcggagtccttggggacggagcagcgcgtcgtggggcgagcggcagaagtcccgggcccagagcccggccagcaggagcagttggtcttcggcagcggggatgctgtggagctgagctgtcccccgcccgggggtggtcccatggggcccactgtctgggtcaaggatggcacagggctggtgccctcggagcgtgtcctggtggggccccagcggctgcaggtgctgaatgcctcccacgaggactccggggcctacagctgccggcagcggctcacgcagcgcgtactgtgccacttcagtgtgcgggtgacagacgctccatcctcgggagatgacgaagacggggaggacgaggctgaggacacaggtgtggacacaggggccccttactggacacggcccgagcggatggacaagaagctgctggccgtgccggccgccaacaccgtccgcttccgctgcccagccgctggcaaccccactccctccatctcctggctgaagaacggcagggagttccgcggcgagcaccgcattggaggcatcaagctgcggcatcagcagtggagcctggtcatggaaagcgtggtgccctcggaccgcggcaactacacctgcgtcgtggagaacaagtttggcagcatccggcagacgtacacgctggacgtgctggagcgctccccgcaccggcccatcctgcaggcggggctgccggccaaccagacggcggtgctgggcagcgacgtggagttccactgcaaggtgtacagtgacgcacagccccacatccagtggctcaagcacgtggaggtgaatggcagcaaggtgggcccggacggcacaccctacgttaccgtgctcaagacggcgggcgctaacaccaccgacaaggagctagaggttctctccttgcacaacgtcacctttgaggacgccggggagtacacctgcctggcgggcaattctattgggttttctcatcactctgcgtggctggtggtgctgccagccgaggaggagctggtggaggctgacgaggcgggcagtgtgtatgcaggcatcctcagctacggggtgggcttcttcctgttcatcctggtggtggcggctgtgacgctctgccgcctgcgcagcccccccaagaaaggcctgggctcccccaccgtgcacaagatctcccgcttcccgctcaagcgacaggtgtccctggagtccaacgcgtccatgagctccaacacaccactggtgcgcatcgcaaggctgtcctcaggggagggccccacgctggccaatgtctccgagctcgagctgcctgccgaccccaaatgggagctgtctcgggcccggctgaccctgggcaagccccttggggagggctgcttcggccaggtggtcatggcggaggccatcggcattgacaaggaccgggccgccaagcctgtcaccgtagccgtgaagatgctgaaagacgatgccactgacaaggacctgtcggacctggtgtctgagatggagatgatgaagatgatcgggaaacacaaaaacatcatcaacctgctgggcgcctgcacgcagggcgggcccctgtacgtgctggtggagtacgcggccaagggtaacctgcgggagtttctgcgggcgcggcggcccccgggcctggactactccttcgacacctgcaagccgcccgaggagcagctcaccttcaaggacctggtgtcctgtgcctaccaggtggcccggggcatggagtacttggcctcccagaagtgcatccacagggacctggctgcccgcaatgtgctggtgaccgaggacaacgtgatgaagatcgcagacttcgggctggcccgggacgtgcacaacctcgactactacaagaagacgaccaacggccggctgcccgtgaagtggatggcgcctgaggccttgtttgaccgagtctacactcaccagagtgacgtctggtcctttggggtcctgctctgggagatcttcacgctggggggctccccgtaccccggcatccctgtggaggagctcttcaagctgctgaaggagggccaccgcatggacaagcccgccaactgcacacacgacctgtacatgatcatgcgggagtgctggcatgccgcgccctcccagaggcccaccttcaagcagctggtggaggacctggaccgtgtccttaccgtgacgtccaccgacgagtacctggacctgtcggcgcctttcgagcagtactccccgggtggccaggacacccccagctccagctcctcaggggacgactccgtgtttgcccacgacctgctgcccccggccccacccagcagtgggggctcgcggacgtgaagggccactggtccccaacaatgtgaggggtccctagcagcccaccctgctgctggtgcacagccactccccggcatgagactcagtgcagatggagagacagctacacagagctttggtctgtgtgtgtgtgtgtgcgtgtgtgtgtgtgtgtgtgcacatccgcgtgtgcctgtgtgcgtgcgcatcttgcctccaggtgcagaggtaccctgggtgtccccgctgctgtgcaacggtctcctgactggtgctgcagcaccgaggggcctttgttctggggggacccagtgcagaatgtaagtgggcccacccggtgggacccccgtggggcagggagctgggcccgacatggctccggcctctgcctttgcaccacgggacatcacagggtgggcctcggcccctcccacacccaaagctgagcctgcagggaagccccacatgtccagcaccttgtgcctggggtgttagtggcaccgcctccccacctccaggctttcccacttcccaccctgcccctcagagactgaaattacgggtacctgaagatgggagcctttaccttttatgcaaaaggtttattccggaaactagtgtacatttctataaatagatgctgtgtatatggtatatatacatatatatatataacatatatggaagaggaaaaggctggtacaacggaggcctgcgaccctgggggcacaggaggcaggcatggccctgggcggggcgtgggggggcgtggagggaggccccagggggtctcacccatgcaagcagaggaccagggccttttctggcaccgcagttttgttttaaaactggacctgtatatttgtaaagctatttatgggcccctggcactcttgttcccacaccccaacacttccagcatttagctggccacatggcggagagttttaatttttaacttattgacaaccgagaaggtttatcccgccgatagagggacggccaagaatgtacgtccagcctgccccggagctggaggatcccctccaagcctaaaaggttgttaatagttggaggtgattccagtgaagatattttatttcctttgtcctttttcaggagaattagatttctataggatttttctttaggagatttattttttggacttcaaagcaagctggtattttcatacaaattcttctaattgctgtgtgtcccaggcagggagacggtttccagggaggggccggccctgtgtgcaggttccgatgttattagatgttacaagtttatatatatctatatatataatttattgagtttttacaagatgtatttgttgtagacttaacacttcttacgcaatgcttctagagttttatagcctggactgctacctttcaaagcttggagggaagccgtgaattcagttggttcgttctgtactgttactgggccctgagtctgggcagctgtcccttgcttgcctgcagggccatggctcagggtggtctcttcttggggcccagtgcatggtggccagaggtgtcacccaaaccggcaggtgcgattttgttaacccagcgacgaactttccgaaaaataaagacacctggttgctaacctg

SEQ ID NO: 140 - DNA, 3950 bp, Homo sapiens
  source 1..3950: mol_type = other DNA
gtcgcgggcagctggcgccgcgcggtcctgctctgccggtcgcacggacgcaccggcgggccgccggccggagggacggggcgggagctgggcccgcggacagcgagccggagcgggagccgcgcgtagcgagccgggctccggcgctcgccagtctcccgagcggcgcccgcctcccgccggtgcccgcgccgggccgtggggggcagcatgcccgcgcgcgctgcctgaggacgccgcggcccccgcccccgccatgggcgcccctgcctgcgccctcgcgctctgcgtggccgtggccatcgtggccggcgcctcctcggagtccttggggacggagcagcgcgtcgtggggcgagcggcagaagtcccgggcccagagcccggccagcaggagcagttggtcttcggcagcggggatgctgtggagctgagctgtcccccgcccgggggtggtcccatggggcccactgtctgggtcaaggatggcacagggctggtgccctcggagcgtgtcctggtggggccccagcggctgcaggtgctgaatgcctcccacgaggactccggggcctacagctgccggcagcggctcacgcagcgcgtactgtgccacttcagtgtgcgggtgacagacgctccatcctcgggagatgacgaagacggggaggacgaggctgaggacacaggtgtggacacaggggccccttactggacacggcccgagcggatggacaagaagctgctggccgtgccggccgccaacaccgtccgcttccgctgcccagccgctggcaaccccactccctccatctcctggctgaagaacggcagggagttccgcggcgagcaccgcattggaggcatcaagctgcggcatcagcagtggagcctggtcatggaaagcgtggtgccctcggaccgcggcaactacacctgcgtcgtggagaacaagtttggcagcatccggcagacgtacacgctggacgtgctggagcgctccccgcaccggcccatcctgcaggcggggctgccggccaaccagacggcggtgctgggcagcgacgtggagttccactgcaaggtgtacagtgacgcacagccccacatccagtggctcaagcacgtggaggtgaatggcagcaaggtgggcccggacggcacaccctacgttaccgtgctcaaggtgtccctggagtccaacgcgtccatgagctccaacacaccactggtgcgcatcgcaaggctgtcctcaggggagggccccacgctggccaatgtctccgagctcgagctgcctgccgaccccaaatgggagctgtctcgggcccggctgaccctgggcaagccccttggggagggctgcttcggccaggtggtcatggcggaggccatcggcattgacaaggaccgggccgccaagcctgtcaccgtagccgtgaagatgctgaaagacgatgccactgacaaggacctgtcggacctggtgtctgagatggagatgatgaagatgatcgggaaacacaaaaacatcatcaacctgctgggcgcctgcacgcagggcgggcccctgtacgtgctggtggagtacgcggccaagggtaacctgcgggagtttctgcgggcgcggcggcccccgggcctggactactccttcgacacctgcaagccgcccgaggagcagctcaccttcaaggacctggtgtcctgtgcctaccaggtggcccggggcatggagtacttggcctcccagaagtgcatccacagggacctggctgcccgcaatgtgctggtgaccgaggacaacgtgatgaagatcgcagacttcgggctggcccgggacgtgcacaacctcgactactacaagaagacgaccaacggccggctgcccgtgaagtggatggcgcctgaggccttgtttgaccgagtctacactcaccagagtgacgtctggtcctttggggtcctgctctgggagatcttcacgctggggggctccccgtaccccggcatccctgtggaggagctcttcaagctgctgaaggagggccaccgcatggacaagcccgccaactgcacacacgacctgtacatgatcatgcgggagtgctggcatgccgcgccctcccagaggcccaccttcaagcagctggtggaggacctggaccgtgtccttaccgtgacgtccaccgacgagtacctggacctgtcggcgcctttcgagcagtactccccgggtggccaggacacccccagctccagctcctcaggggacgactccgtgtttgcccacgacctgctgcccccggccccacccagcagtgggggctcgcggacgtgaagggccactggtccccaacaatgtgaggggtccctagcagcccaccctgctgctggtgcacagccactccccggcatgagactcagtgcagatggagagacagctacacagagctttggtctgtgtgtgtgtgtgtgcgtgtgtgtgtgtgtgtgtgcacatccgcgtgtgcctgtgtgcgtgcgcatcttgcctccaggtgcagaggtaccctgggtgtccccgctgctgtgcaacggtctcctgactggtgctgcagcaccgaggggcctttgttctggggggacccagtgcagaatgtaagtgggcccacccggtgggacccccgtggggcagggagctgggcccgacatggctccggcctctgcctttgcaccacgggacatcacagggtgggcctcggcccctcccacacccaaagctgagcctgcagggaagccccacatgtccagcaccttgtgcctggggtgttagtggcaccgcctccccacctccaggctttcccacttcccaccctgcccctcagagactgaaattacgggtacctgaagatgggagcctttaccttttatgcaaaaggtttattccggaaactagtgtacatttctataaatagatgctgtgtatatggtatatatacatatatatatataacatatatggaagaggaaaaggctggtacaacggaggcctgcgaccctgggggcacaggaggcaggcatggccctgggcggggcgtgggggggcgtggagggaggccccagggggtctcacccatgcaagcagaggaccagggccttttctggcaccgcagttttgttttaaaactggacctgtatatttgtaaagctatttatgggcccctggcactcttgttcccacaccccaacacttccagcatttagctggccacatggcggagagttttaatttttaacttattgacaaccgagaaggtttatcccgccgatagagggacggccaagaatgtacgtccagcctgccccggagctggaggatcccctccaagcctaaaaggttgttaatagttggaggtgattccagtgaagatattttatttcctttgtcctttttcaggagaattagatttctataggatttttctttaggagatttattttttggacttcaaagcaagctggtattttcatacaaattcttctaattgctgtgtgtcccaggcagggagacggtttccagggaggggccggccctgtgtgcaggttccgatgttattagatgttacaagtttatatatatctatatatataatttattgagtttttacaagatgtatttgttgtagacttaacacttcttacgcaatgcttctagagttttatagcctggactgctacctttcaaagcttggagggaagccgtgaattcagttggttcgttctgtactgttactgggccctgagtctgggcagctgtcccttgcttgcctgcagggccatggctcagggtggtctcttcttggggcccagtgcatggtggccagaggtgtcacccaaaccggcaggtgcgattttgttaacccagcgacgaactttccgaaaaataaagacacctggttgctaacctg

SEQ ID NO: 141 - DNA, 2085 bp, Homo sapiens
  source 1..2085: mol_type = other DNA
atgggcgcccctgcctgcgccctcgcgctctgcgtggccgtggccatcgtggccggcgcctcctcggagtccttggggacggagcagcgcgtcgtggggcgagcggcagaagtcccgggcccagagcccggccagcaggagcagttggtcttcggcagcggggatgctgtggagctgagctgtcccccgcccgggggtggtcccatggggcccactgtctgggtcaaggatggcacagggctggtgccctcggagcgtgtcctggtggggccccagcggctgcaggtgctgaatgcctcccacgaggactccggggcctacagctgccggcagcggctcacgcagcgcgtactgtgccacttcagtgtgcgggtgacagacgctccatcctcgggagatgacgaagacggggaggacgaggctgaggacacaggtgtggacacaggggccccttactggacacggcccgagcggatggacaagaagctgctggccgtgccggccgccaacaccgtccgcttccgctgcccagccgctggcaaccccactccctccatctcctggctgaagaacggcagggagttccgcggcgagcaccgcattggaggcatcaagctgcggcatcagcagtggagcctggtcatggaaagcgtggtgccctcggaccgcggcaactacacctgcgtcgtggagaacaagtttggcagcatccggcagacgtacacgctggacgtgctggagcgctccccgcaccggcccatcctgcaggcggggctgccggccaaccagacggcggtgctgggcagcgacgtggagttccactgcaaggtgtacagtgacgcacagccccacatccagtggctcaagcacgtggaggtgaacggcagcaaggtgggcccggacggcacaccctacgttaccgtgctcaaggtgtccctggagtccaacgcgtccatgagctccaacacaccactggtgcgcatcgcaaggctgtcctcaggggagggccccacgctggccaatgtctccgagctcgagctgcctgccgaccccaaatgggagctgtctcgggcccggctgaccctgggcaagccccttggggagggctgcttcggccaggtggtcatggcggaggccatcggcattgacaaggaccgggccgccaagcctgtcaccgtagccgtgaagatgctgaaagacgatgccactgacaaggacctgtcggacctggtgtctgagatggagatgatgaagatgatcgggaaacacaaaaacatcatcaacctgctgggcgcctgcacgcagggcgggcccctgtacgtgctggtggagtacgcggccaagggtaacctgcgggagtttctgcgggcgcggcggcccccgggcctggactactccttcgacacctgcaagccgcccgaggagcagctcaccttcaaggacctggtgtcctgtgcctaccaggtggcccggggcatggagtacttggcctcccagaagtgcatccacagggacctggctgcccgcaatgtgctggtgaccgaggacaacgtgatgaagatcgcagacttcgggctggcccgggacgtgcacaacctcgactactacaagaagacaaccaacggccggctgcccgtgaagtggatggcgcctgaggccttgtttgaccgagtctacactcaccagagtgacgtctggtcctttggggtcctgctctgggagatcttcacgctggggggctccccgtaccccggcatccctgtggaggagctcttcaagctgctgaaggagggccaccgcatggacaagcccgccaactgcacacacgacctgtacatgatcatgcgggagtgctggcatgccgcgccctcccagaggcccaccttcaagcagctggtggaggacctggaccgtgtccttaccgtgacgtccaccgacgagtacctggacctgtcggcgcctttcgagcagtactccccgggtggccaggacacccccagctccagctcctcaggggacgactccgtgtttgcccacgacctgctgcccccggccccacccagcagtgggggctcgcggacgtga

SEQ ID NO: 142 - DNA, 4431 bp, Homo sapiens
  source 1..4431: mol_type = other DNA
aggcggggctggagtggtggaaggggggtggcaggtctgcattgccgcttccctggtgccgggagcagtcgccgctgccgcctccgcccgcggccgggacccccgtcctcgcccgggactccttacccggggaacctagaccaggtctccagaggcttgtggaagagaagcaggcgacccttcctgagttatcctggcttagcctcccaatctggctccccttccccttcccattcccctgctccccctgtcccttccccatccacccaactgaactgggtataggtcaaagctcctctctttccttttccttcctaggcactcattggctaggacctgtttgctcttttttttgtgcccagagatactggaacacgcttcatctaagtaactgtggggaggggtctttttgactctacaagtccttgagcaaaaagctgaaaaagaagcaggaggtggagaagacccagtgaagtgccccaagccccatcatggaagagggcttccgagaccgggcagctttcatccgtggggccaaagacattgctaaggaagtcaaaaagcatgcggccaagaaggtggtgaagggcctggacagagtccaggacgaatattcccgaagatcgtactcccgctttgaggaggaggatgatgatgatgacttccctgctcccagtgatggttattaccgaggagaagggacccaggatgaggaggaaggtggtgcatccagtgatgctactgagggccatgacgaggatgatgagatctatgaaggggaatatcagggcattccccgggcagagtctgggggcaaaggcgagcggatggcagatggggcgcccctggctggagtaagggggggcttgagtgatggggagggtccccctgggggccggggggaggcacaacgacggaaagaacgagaagaactggcccaacagtatgaagccatcctacgggagtgtggccacggccgcttccagtggacactgtattttgtgcttggtctggcgctgatggctgacggtgtggaggtctttgtggtgggcttcgtgctgcccagcgctgagaaagacatgtgcctgtccgactccaacaaaggcatgctaggcctcatcgtctacctgggcatgatggtgggagccttcctctggggaggtctggctgaccggctgggtcggaggcagtgtctgctcatctcgctctcagtcaacagcgtcttcgccttcttctcatcttttgtccagggttacggcactttcctcttctgccgcctactttctggggttgggattggagggtccatccccattgtcttctcctatttctccgagtttctggcccaggagaaacgaggggagcatttgagctggctctgcatgttttggatgattggtggcgtgtacgcagctgctatggcctgggccatcatcccccactatgggtggagttttcagatgggttctgcctaccagttccacagctggagggtcttcgtcctcgtctgcgcctttccttctgtgtttgccattggggctctgaccacgcagcctgagagcccccgtttcttcctagagaatggaaagcatgatgaggcctggatggtgctgaagcaggtccatgataccaacatgcgagccaaaggacatcctgagcgagtgttctcagtaacccacattaagacgattcatcaggaggatgaattgattgagatccagtcggacacagggacctggtaccagcgctggggggtccgggccttgagcctaggggggcaggtttgggggaattttctctcctgttttggtcccgaatatcggcgcatcactctgatgatgatgggtgtgtggttcaccatgtcattcagctactatggcctgaccgtctggtttcctgacatgatccgccatctccaggcagtggactacgcatcccgcaccaaagtgttccccggggagcgcgtagagcatgtaacttttaacttcacgttggagaatcagatccaccgaggcgggcagtacttcaatgacaagttcattgggctgcggctcaagtcagtgtcctttgaggattccctgtttgaagagtgttattttgaggatgtcacatccagcaacacgtttttccgcaactgcacattcatcaacactgtgttctataacactgacctgttcgagtacaagtttgtgaacagccgtctgataaacagtacattcctgcacaacaaggagggctgcccgctagacgtgacagggacgggcgaaggtgcctacatggtatactttgtgagcttcctggggacactggcagtgcttcctgggaatatcgtgtctgccctgctcatggacaagatcggcaggctcagaatgcttgctggctccagcgtgatgtcctgtgtctcctgcttcttcctgtcttttgggaacagtgagtcggccatgatcgctctgctctgcctttttggcggggtcagcattgcatcctggaatgcgctggacgtgttgactgttgaactctacccctcagacaagaggaccacagcttttggcttcctgaatgccctgtgtaagctggcagctgtgctggggatcagcatcttcacatccttcgtgggaatcaccaaggctgcacccatcctctttgcctcagctgcccttgcccttggcagctctctggccctgaagctgcctgagacccgggggcaggtgctgcagtgaaggggtctctagggctttgggattggcaggcacactgtgagaccaacaactccttccttcccctccctgccctgccatcctgacctccagagccctcactccccactccccgtgtttggtgtcttagctgtgtgtgcgtgtgcgtgtgcatgtgtgtaaaccccgtgggcagggactacagggaaggctccttcatcccagttttgagatgaagctgtactccccatttcccactgcccttgactttgcacaagagaaggctgagccccatccttctccccctgttagagaggggcccttgcttccctgttccaggggttccagaataggcttcctgccttccccatcattccctctgcctaggccctggtgaaaccacaggtatgcaattatgctaggggctggggctctggtgtagaccatggaccaaaagaacttcttagagtctgaagagtgggcctcgggtgccctctcacatctcctgttggatgctgggggagaagcaataaacctcagccctctggcctccactttcctctcaatttgggctgcaaatatgaagcctgaattttatgaaattagctttctgattcttatttattaatagattaagttctgaggcagctccgcaggactgtgtgtgaatgtgtatgtatacttacatatgtgtgtgcatgtgccatggggcggggggtatcactatactgtcctcaaatataagccaagggtaatttcagcggatgcacacacaaccctgcctcccacagttcctcccctaatctggtttctgtgttgagcctgggatggaggagccctaggccagcctgggataagagtcccacagtctagggagatctgagggcatccgacaaggcccatctccttccctcctcaagaagcagaggcctcctctggagtgagaggctccacccactacagcacaggcgggaatagcacagctgccctcccatgctccctacctgtcccctcacagggaggggagcaggggagggaaagaaaccaggcatctggtcaaaccagcagatcaaaaagcacaaagagctggggcagaggcaggaagcaggggccctcctggcagctcctctgagtggggagaggttgggcagtgagtgagggacccctaatgcagggactagaagcctcagtttccccattttacccttccacacaatagcctctgtaggttaggctgccccatcccaccctactctgtgtggctgctttctttggtgccctcccctcaccccactgtagctgtgacgtgttgtagtttttagatgtttgtaaaatgtttaaaaaaatgttaaaaggaaaaaagtgaaaataacaaaaaagaaaatcaaaattcaccttcgtcatgctgcgtccagtgccccaaccctgtggtcactctccccattttgtaacactgtaccaggtggtgactgtttaactctttggtgtctgtgctcaaaagactgccttctccagtgcccagtgtatgagtgtgtgccctgtgcccttgtccctcactccccacatgctggacgtagccctcttcctcgcacccctgggagggacccatccatctcccttgctctcctggggaaccctaaacccaactctgttgatgtgaaaaatgcagtgaaaaatattgacgaaaaataaaacggaaacaaatcctcaaaatacaaaaaaaaaaaaaaaaaaa

SEQ ID NO: 143 - DNA, 5311 bp, Homo sapiens
  source 1..5311: mol_type = other DNA
agcataaccttcggtggcaggacaaatcaggccagcacgcagtctgccaagtcctgctcgctccctgtcaagaaaaacagctggatccatttctaatcaacacttcccaacgcaacacttctgagtctctgaaggagaccagagcttgaaactttccagacttccaacagacatcgagtgcaaaaggatatttaggttgtctttgcacaaatctggttgatttgagagataaagggggggggaaccagtgtgactttcacctaagaagtcacatgaacatatttcacatttgaactacataatgaatgatggttattgaaatagcccaaacctctaccacagagcgagggatatagctcaaggggcaaccaggcagtcgcagaaccaaggaatggatgactacaagtatcaggacaattatgggggctatgctcccagtgatggctattaccgcggcaatgagtccaacccagaagaagatgcacagagtgatgtcaccgaaggccatgatgaggaagacgagatctatgagggcgagtaccagggtatccctcacccagatgatgtcaaggccaagcaggccaagatggcgccctccagaatggacagccttcggggccagacagacctgatggctgagaggctggaagatgaggagcagttggcccaccagtacgagaccatcatggatgagtgtggccatggccgcttccagtggatcctctttttcgtcttgggtttggccctgatggccgatggggtggaagtgttcgtggtgagttttgccctgcccagtgcagagaaggacatgtgtctgtccagttccaaaaaaggaatgctagggatgatagtctacttgggaatgatggcgggcgccttcatcctgggaggcctggctgataagctgggaaggaagcgagtcctcagcatgtctctggccgtcaatgcctccttcgcctccctctcttccttcgtgcagggatatggagccttcctcttctgccgactcatctcaggcatcggtattgggggtgctctaccgattgtttttgcctatttttctgaattcttgtctcgggagaagcgaggagaacacctcagttggctgggcatcttctggatgactgggggcctgtacgcatctgccatggcctggagcatcatcccacactatggctggggcttcagcatggggaccaattaccacttccatagctggagagtgtttgtcatcgtctgtgctctgccctgcaccgtgtccatggtggccctgaagttcatgccagagagcccaaggtttctgctagagatgggcaaacatgatgaagcctggatgattctcaagcaagtccatgacaccaacatgagagctaaggggaccccagagaaagtgttcacggtttccaacatcaaaactcccaagcaaatggatgaattcattgagatccaaagttcaacaggaacctggtaccagcgctggctggtcagattcaagaccattttcaagcaggtctgggataatgccctgtactgtgtgatggggccctacagaatgaatacactgattctggccgtggtttggtttgccatggcattcagttactatggactgacagtttggtttcctgatatgatccgctattttcaagatgaagaatacaagtctaaaatgaaggtgttttttggtgagcatgtgtacggcgccacaatcaacttcacgatggaaaatcagatccaccaacatgggaaacttgtgaatgataagttcacaagaatgtactttaaacatgtactctttgaggacacattctttgacgagtgctattttgaagacgtaacatcaacagatacctacttcaaaaattgtaccattgaatcaaccatcttttacaacacagacctctacgagcacaagttcatcaactgtcggtttatcaactccaccttcctggagcagaaggagggctgccacatggacttggagcaagataatgacttcctgatttacctcgtcagcttcctgggcagcctgtctgtcttacccgggaacatcatttctgccctgctcatggatagaattggaaggctcaagatgattggtggctccatgctaatctctgcagtctgctgcttcttcctgttttttggcaacagtgagtctgcaatgatcggctggcagtgcctgttctgtgggacaagcattgcagcctggaatgctctggatgtgatcacagtggagctgtatcccaccaaccagagagcaacagccttcggcattctcaatggattatgcaaatttggcgccatcctgggaaacaccatctttgcttcttttgttgggataaccaaagtggtccccatccttctggctgctgcttctctggttgggggtggcctgattgcccttcgactgccagagactcgagaacaggtcctgatgtgaacaacctatgggaaaaggaaaggtcgagagaatcttgtccaggacactgaaatgcatccacacttcctgcctatcacggtccggaggacaccttggatagcacgggaggagaagttgactttgtgacccctagtttaggacccacttcagctgtcaatatgtttgtaactcaggtgactgatttgggggtgccctgagccacccttagaatcacagagctgcgtgtttaacttcaagtcttcccagtccaaggcagggagaggattctccagtgagtgcacacactatgcgaggagcaagcatttctctaagtcaagtgcaaggacttaacttgcgtttgaaaaggaattagagggtcagaaacacccaggttcctccagaaagctccttggagcccaacaacttaacaaatcaacttggctggaagttagagtcattatatgaagattgggcttgaagtatatatttttgcatttaaaagtatcacctatcatattttccactcgaaaattgacatagtagcattgaggatactctgatctagaaagccaagtatttgagcaacatctatagagatctacttttctcctatgtctcctaggctttccatgataattaggtaatacatttaagaaggatatttatttctgttttgctctattcaaagaaacggaatgggatagttattctgtaaactaagtttgtatataactttatttgggtttaatttccacaactggtatctgcaaatattgccagcattttagccatattttgggagaacttggtgtttgaggtcccaggaaatgaggtctgatcaaatgaaatgcaagcacaatttcttacagccatttaactttctgttgggaggatgaattaacaaactcacattgtgcagtctgcttaatccaggcacttttctttgtgcaggtgtagtgagtagttacttctctcccttacacagatgacttgtgaaactcaagctcaccatcttcagtgctggcattttactttgccactacccaaaaacaatgtgagatgtgttcagtggcctctggtactctttgcaggcaagaatcaaacaacatggggactgagggaaggatggggaagtgtagccacagttcttccaaatgtaaatactttttgtttgttctagtggtaaaatgcaaatgcaatccatatttgttaggatggtcaggtctcatgagaaatctatgctatgtgtccagagcttttgaaacagagtccattggagtgggagttagggagtgtagtggatgccaaatatgtttttcttcagtgcttaagagaactgtttcctgaagtccagctttgaacataaacaggggtgtgggttgggggaggagcttaggacaaacctctctgatgaaggtcagcaatagactgaagtcttgactgcatggaagaggaaaaacatcagaactgtctgacaatggaggggacagtgagctacgcacaactgccagcggaggtgaacttgcacctgcccaggccggatgaacatcagcctgcaagaactagttgtttgagttgatttgcagtgctctcaatgggcaagtgccacattttccctggcagagatctccaaaaatttaaaacagaataataatggctatatcgagtgttttctcagtattggagaaatgcttaggtcctatgatagcttcgggacatctttctgtaattttcctcaattaacgggttggtaggggtaaatcttatgacacctttccaccgtcgatttgagatcagttttaatggttaaaatgtttactctccttctgtcaaccctcacctttttatttacacccctccctttttttctgtacagggagagaagacatattgactctgactggacaccctgattcctccaaatatatataccactgtgtattaatctttctctcagtgttttataggagtactaacatttattgctctgtcaataatgaaaggctcgatgtaatatagctgtaatttactttccatatgaatacagtggctaggttcataaaagagaattgtgtgagtctgggattaccacatctaaaacattattctttaatgggataatacaattcattgagcagctaccacttaaaaaacttgcaggacagttagagcctgcatttctagttaagatggatcttgtaaatttaaaattggattaacattggagtgctggggtggctgcaataatttgggggctaactccatttggtttccaagatctcacttctgcattatctttatggctctttaaaccagccacctagccaatcaagggcaattcccatctcatccatcactcaggtctttgtaaagggtgcagccaagctctgcagacttttgcaggattgtctagcctgagtaccgggctacttcttaaatgccgtcactcctgctgagataaatgcgtctttaaaaatagtctctgtggcaggtcactgggggacaatgtacagcattctggccatccacttctttttcacttcatgttctaccccaagagactcccgatgtcggctgtggagggttaaagggatgaggctttcctttgtttagcaaatctgttcacagttcttgatgatgtattttatgatgcccagcttggaaatagttgctttccatagtctcaactgtattgtgtcatctcctgatgctgatttttgatcttttgttttattaaaaataattagtgaaagaggtgtgcctatctgtgaagtttgtagtacatcatcctgaggtcatgtaacaagtaaaccccaacccagcgttccctcctacgttgtgttagttcattaaaactaaataataaaaataactgtaagaaaaccttaa

SEQ ID NO: 144 - DNA, 2362 bp, Homo sapiens
  source 1..2362: mol_type = other DNA
cactcagggcaagggtgtccgacggctggagcgttctgttttgaacccaaagtggatgatgctgtcagagctgaactactgaaaggaggctgtgaaaatttcccatcttctcattggccatcagttgagataagatggaagactcttacaaggataggacttcactgatgaagggtgccaaggacattgccagagaggtgaagaaacaaacagtaaagaaggtgaatcaagctgtggaccgagcccaggatgaatacacccagaggtcctacagtcggttccaagatgaagaagatgatgatgactactacccggctggagaaacctataatggtgaggccaacgatgacgaaggctcaagtgaagccactgaggggcatgatgaagatgatgagatctatgagggggagtatcagggcatccccagtatgaaccaagcgaaggacagcatcgtgtcagtggggcagcccaagggcgatgagtacaaggaccgacgggagctggaatcagaaaggagagctgacgaggaagagttagcccagcagtatgagctgataatccaagaatgcggtcatggtcgttttcagtgggcccttttcttcgtcctgggcatggctcttatggcagacggtgtagaggtgtttgtcgttggcttcgtgttacccagtgctgagacagacctctgcatcccaaattcaggatctggatggctaggcagcatagtgtacctcgggatgatggtgggggcgttcttctggggaggactggcagacaaagtgggaaggaaacagtctcttctgatttgcatgtctgtcaacggattctttgccttcctttcttcatttgtccaaggttatggcttctttctcttctgtcgcttactttctggattcgggattggaggagccatacccactgtgttctcgtactttgctgaagtcctggcccgggaaaagcggggcgaacacttgagctggctctgcatgttctggatgatcggtggcatctacgcctctgccatggcctgggccatcatcccgcactacgggtggagcttcagcatgggatcggcctaccagtttcacagttggcgtgtgtttgtcatcgtctgtgcactcccctgtgtctcctccgtggtggccctcacattcatgcctgaaagcccacgattcttgttggaggttggaaaacatgatgaagcttggatgattctgaagttaattcatgacaccaacatgagagcccggggtcagcctgagaaggtcttcacggtaaacaaaataaaaactcctaaacaaatagatgagctgattgaaattgagagtgacacaggaacatggtataggaggtgttttgttcggatccgcaccgagctgtacggaatttggttgacttttatgagatgtttcaactacccagtcagggataatacaataaagcttacaattgtttggttcaccctgtcctttgggtactatggattatccgtttggttccctgatgtcattaaacctctgcagtccgatgaatatgcattgctaaccagaaatgtggagagagataaatatgcaaatttcactattaactttacaatggaaaatcagattcatactggaatggaatacgacaatggcagattcataggggtcaagttcaaatctgtaactttcaaagactctgtttttaagtcctgcacctttgaggatgtaacttcagtgaacacctacttcaagaactgcacatttattgacactgtttttgacaacacagattttgagccatataaattcattgacagtgaatttaaaaactgctcgttttttcacaacaagacgggatgtcagattacctttgatgatgactatagtgcctactggatttattttgtcaactttctggggacattggcagtattgccagggaacattgtgtctgctctgctgatggacagaattgggcgcttaacaatgctaggtggctctatggtgctttcggggatcagctgtttcttcctttggttcggcaccagtgaatccatgatgataggcatgctgtgtctgtacaatggattgaccatctcagcctggaactctcttgacgtggtcactgtggaactgtaccccacagaccggagggcaacaggctttggcttcttaaatgcgctatgcaaggcagcagccgtcctgggaaacttaatatttggctctctggtcagcatcaccaaatcaatccccatcctgctggcttctactgtgctcgtgtgtggaggactcgttgggctgtgcctgcctgacacacgaacccaggttctgatgtaatgggaaaaaaagccatccttcctgcgtttcttcctcctgccctg

SEQ ID NO: 145 - DNA, 2053 bp, Homo sapiens
  source 1..2053: mol_type = other DNA
catctttgatgagggcagagctcacgttgcattgaagacgaaacctcggggaggtcaggcgctgtctttccttccctccctgctcggcggctccaccacagttgcaacctgcagaggcccggagaacacaaccctcccgagaagcccaggtccagagccaaacccgtcactgaccccccagcccaggcgcccagccactccccaccgctaccatggccgaagacgcagacatgcgcaatgagctggaggagatgcagcgaagggctgaccagttggctgatgagtcgctggaaagcacccgtcgtatgctgcaactggttgaagagagtaaagatgctggtatcaggactttggttatgttggatgaacaaggagaacaactcgatcgtgtcgaagaaggcatgaaccatatcaaccaagacatgaaggaggctgagaaaaatttaaaagatttagggaaatgctgtggccttttcatatgtccttgtaacaagcttaaatcaagtgatgcttacaaaaaagcctggggcaataatcaggacggagtggtggccagccagcctgctcgtgtagtggacgaacgggagcagatggccatcagtggcggcttcatccgcagggtaacaaatgatgcccgagaaaatgaaatggatgaaaacctagagcaggtgagcggcatcatcgggaacctccgtcacatggccctggatatgggcaatgagatcgatacacagaatcgccagatcgacaggatcatggagaaggctgattccaacaaaaccagaattgatgaggccaaccaacgtgcaacaaagatgctgggaagtggttaagtgtgcccacccgtgttctcctccaaatgctgtcgggcaagatagctccttcatgcttttctcatggtattatctagtaggtctgcacacataacacacatcagtccacccccattgtgaatgttgtcctgtgtcatctgtcagcttcccaacaatactttgtgtcttttgttctctcttggtctctttctttccaaaggttgtacatagtggtcatttggtggctctaactccttgatgtcttgagtttcatttttcattttctctcctcggtggcatttgctgaataacaacaatttaggaatgctcaatgtgctgttgattctttcaatccacagtattgttcttgtaaaactgtgacattccacagagttactgccacggtcctttgagtgtcaggctctgaatctctcaaaatgtgccgtctttggttcctcatggctgttatctgtctttatgatttcatgattagacaatgtggaattacataacaggcattgcactaaaagtgatgtgatttatgcatttatgcatgagaactaaatagatttttagattcctacttaaacaaaaactttccatgacagtagcatactgatgagacaacacacacacacacaaaacaacagcaacaacaacagaacaacaacaaagcatgctcagtattgagacactgtcaagattaagttataccagcaaaagtgcagtagtgtcacttttttcctgtcaatatatagagacttctaaatcataatcatccttttttaaaaaaaagaattttaaaaaagatggatttgacacactcaccatttaatcatttccagcaaaatatatgtttggctgaaattatgtcaaatggatgtaatatagggtttgtttgctgcttttgatggctacgttttggagagagcaatcttgctgtgaaacagtgtggatgtaaattttataaggctgactcttactaaccaccatttcccctgtggtttgttatcagtacaattctttgttgcttaatctagagctatgcacaccaaattgctgagatgtttagtagctgataaagaaaccttttaaaaaaataatataaatgaatgaaatataaactgtgagataaatatcattatagcatgtaatattaaattcctcctgtctcctctgtcagtttgtgaagtgattgacattttgtagctagtttaaaattattaaaaattatagactcc

SEQ ID NO: 146 - DNA, 2053 bp, Homo sapiens
  source 1..2053: mol_type = other DNA
catctttgatgagggcagagctcacgttgcattgaagacgaaacctcggggaggtcaggcgctgtctttccttccctccctgctcggcggctccaccacagttgcaacctgcagaggcccggagaacacaaccctcccgagaagcccaggtccagagccaaacccgtcactgaccccccagcccaggcgcccagccactccccaccgctaccatggccgaagacgcagacatgcgcaatgagctggaggagatgcagcgaagggctgaccagttggctgatgagtcgctggaaagcacccgtcgtatgctgcaactggttgaagagagtaaagatgctggtatcaggactttggttatgttggatgaacaaggagaacaactggaacgcattgaggaagggatggaccaaatcaataaggacatgaaagaagcagaaaagaatttgacggacctaggaaaattctgcgggctttgtgtgtgtccctgtaacaagcttaaatcaagtgatgcttacaaaaaagcctggggcaataatcaggacggagtggtggccagccagcctgctcgtgtagtggacgaacgggagcagatggccatcagtggcggcttcatccgcagggtaacaaatgatgcccgagaaaatgaaatggatgaaaacctagagcaggtgagcggcatcatcgggaacctccgtcacatggccctggatatgggcaatgagatcgatacacagaatcgccagatcgacaggatcatggagaaggctgattccaacaaaaccagaattgatgaggccaaccaacgtgcaacaaagatgctgggaagtggttaagtgtgcccacccgtgttctcctccaaatgctgtcgggcaagatagctccttcatgcttttctcatggtattatctagtaggtctgcacacataacacacatcagtccacccccattgtgaatgttgtcctgtgtcatctgtcagcttcccaacaatactttgtgtcttttgttctctcttggtctctttctttccaaaggttgtacatagtggtcatttggtggctctaactccttgatgtcttgagtttcatttttcattttctctcctcggtggcatttgctgaataacaacaatttaggaatgctcaatgtgctgttgattctttcaatccacagtattgttcttgtaaaactgtgacattccacagagttactgccacggtcctttgagtgtcaggctctgaatctctcaaaatgtgccgtctttggttcctcatggctgttatctgtctttatgatttcatgattagacaatgtggaattacataacaggcattgcactaaaagtgatgtgatttatgcatttatgcatgagaactaaatagatttttagattcctacttaaacaaaaactttccatgacagtagcatactgatgagacaacacacacacacacaaaacaacagcaacaacaacagaacaacaacaaagcatgctcagtattgagacactgtcaagattaagttataccagcaaaagtgcagtagtgtcacttttttcctgtcaatatatagagacttctaaatcataatcatccttttttaaaaaaaagaattttaaaaaagatggatttgacacactcaccatttaatcatttccagcaaaatatatgtttggctgaaattatgtcaaatggatgtaatatagggtttgtttgctgcttttgatggctacgttttggagagagcaatcttgctgtgaaacagtgtggatgtaaattttataaggctgactcttactaaccaccatttcccctgtggtttgttatcagtacaattctttgttgcttaatctagagctatgcacaccaaattgctgagatgtttagtagctgataaagaaaccttttaaaaaaataatataaatgaatgaaatataaactgtgagataaatatcattatagcatgtaatattaaattcctcctgtctcctctgtcagtttgtgaagtgattgacattttgtagctagtttaaaattattaaaaattatagactcc

SEQ ID NO: 147 - protein, 5 aa, synthetic construct
  REGION 1..5: note = SNAP-25 antigen having a free carboxyl-terminus atthe P1 residue of the scissile bond of the BoNT/Acleavage site
DEANQ

SEQ ID NO: 148 - protein, 6 aa, synthetic construct
  REGION 1..6: note = SNAP-25 antigen having a free carboxyl-terminus atthe P1 residue of the scissile bond of the BoNT/Acleavage site
IDEANQ